European Patent Specification EP 3 504 225 B1, published April 24, 2024. Title: NOVEL MAMMALIAN EXPRESSED HUMAN IMMUNODEFICIENCY VIRUS ENVELOPE PROTEIN ANTIGENS. Applicant: GRIFOLS DIAGNOSTIC SOLUTIONS INC. The sequence listing filed with the application follows.

SEQUENCE LISTING (111 sequences)

SEQ ID NO: 1 - protein, 538 aa, Synthetic
MYRMQLLSCIALSLALVTNSNMWKNDMVEQMHEDIISLWCTDLKNDTNTNSSSGRMIMEKAEAAAKEAAAKATSIRGKVQKEYAFFYKLDIIPIDNDTTSYKLTSCAEAAAKEAAAKAPIPIHYCAPAGFAILKCNNKTFNGTGPCTNVSTVCTRPNNNTRKRIRIQRGPGRAFVTIAEAAAKEAAAKAFGNNKTIIFKQSSGGDAEAAAKEAAAKAAEAAAKEAAAKAPCRIKQIINMWQKVGKAMYAPPISGQIAEAAAKEAAAKALTRDGGNSNNESEIFRPGGGDAEAAAKEAAAKAIEPLGVAPTKAKRRVVQREKAPNLLGGPSVFIFPPKIKDVLMISLSPIVTCVVVDVSEDDPDVQISWFVNNVEVHTAQTQTHREDYNSTLRVVSALPIQHQDWMSGKEFKCKVNNKDLPAPIERTISKPKGSVRAPQVYVLPPPEEEMTKKQVTLTCMVTDFMPEDIYVEWTNNGKTELNYKNTEPVLDSDGSYFMYSKLRVEKKNWVERNSYSCSVVHEGLHNHHTTKSFSRTPGK

SEQ ID NO: 2 - protein, 604 aa, Synthetic
MYRMQLLSCIALSLALVTNSTWIQNPGTKWYQNPGTKIYTCTDLKNDTNTNSSSGRMIMEKTWIQNPGTKWYQNPGTKIYTTSIRGKVQKEYAFFYKLDIIPIDNDTTSYKLTSCTWIQNPGTKWYQNPGTKIYTPIPIHYCAPAGFAILKCNNKTFNGTGPCTNVSTVTWIQNPGTKWYQNPGTKIYTCTRPNNNTRKRIRIQRGPGRAFVTITWIQNPGTKWYQNPGTKIYTFGNNKTIIFKQSSGGDTWIQNPGTKWYQNPGTKIYTPCRIKQIINMWQKVGKAMYAPPISGQIAEAAAKEAAAKALTRDGGNSNNESEIFRPGGGDAEAAAKEAAAKAIEPLGVAPTKAKRRVVQREKRGGGPSNMWKNDMVEQMHEDIISLWAPNLLGGPSVFIFPPKIKDVLMISLSPIVTCVVVDVSEDDPDVQISWFVNNVEVHTAQTQTHREDYNSTLRVVSALPIQHQDWMSGKEFKCKVNNKDLPAPIERTISKPKGSVRAPQVYVLPPPEEEMTKKQVTLTCMVTDFMPEDIYVEWTNNGKTELNYKNTEPVLDSDGSYFMYSKLRVEKKNWVERNSYSCSVVHEGLHNHHTTKSFSRTPGK

SEQ ID NO: 3 - protein, 535 aa, Synthetic
MYRMQLLSCIALSLALVTNSNMWKNDMVEQMHEDIISLWCTDLKNDTNTNSSSGRMIMEKAEAAAKEAAAKATSIRGKVQKEYAFFYKLDIIPIDNDTTSYKLTSCAEAAAKEAAAKAPIPIHYCAPAGFAILKCNNKTFNGTGPCTNVSTVCTRPNNNTRKRIRIQRGPGRAFVTIAEAAAKEAAAKAFGNNKTIIFKQSSGGDAEAAAKEAAAKAAEAAAKEAAAKAPCRIKQIINMWQKVGKAMYAPPISGQIAEAAAKEAAAKALTRDGGNSNNESEIFRPGGGDAEAAAKEAAAKAIEPLGVAPTKAKRRVVQREKVPEVSSVFIFPPKPKDVLTITLTPKVTCVVVDISKDDPEVQFSWFVDDVEVHTAQTQPREEQFNSTFRSVSELPIMHQDWLNGKEFKCRVNSAAFPAPIEKTISKTKGRPKAPQVYTIPPPKEQMAKDKVSLTCMITDFFPEDITVEWQWNGQPAENYKNTQPIMDTDGSYFVYSKLNVQKSNWEAGNTFTCSVLHEGLHNHHTEKSLSHSPGI

SEQ ID NO: 4 - protein, 606 aa, Synthetic
MYRMQLLSCIALSLALVTNSTWIQNPGTKWYQNPGTKIYTCTDLKNDTNTNSSSGRMIMEKTWIQNPGTKWYQNPGTKIYTTSIRGKVQKEYAFFYKLDIIPIDNDTTSYKLTSCTWIQNPGTKWYQNPGTKIYTPIPIHYCAPAGFAILKCNNKTFNGTGPCTNVSTVTWIQNPGTKWYQNPGTKIYTCTRPNNNTRKRIRIQRGPGRAFVTITWIQNPGTKIYTFGNNKTIIFKQSSGGDTWIQNPGTKWYQNPGTKIYTPCRIKQIINMWQKVGKAMYAPPISGQIAEAAAKEAAAKALTRDGGNSNNESEIFRPGGGDAEAAAKEAAAKAIEPLGVAPTKAKRRVVQREKRGGGPSNMWKNDMVEQMHEDIISLWVPRDCGCKPCICTVPEVSSVFIFPPKPKDVLTITLTPKVTCVVVDISKDDPEVQFSWFVDDVEVHTAQTQPREEQFNSTFRSVSELPIMHQDWLNGKEFKCRVNSAAFPAPIEKTISKTKGRPKAPQVYTIPPPKEQMAKDKVSLTCMITDFFPEDITVEWQWNGQPAENYKNTQPIMDTDGSYFVYSKLNVQKSNWEAGNTFTCSVLHEGLHNHHTEKSLSHSPGI

SEQ ID NO: 5 - protein, 378 aa, Synthetic
MYRMQLLSCIALSLALVTNSNMWKNDMVEQMHEDIISLWCTDLKNDTNTNSSSGRMIMEKAEAAAKEAAAKATSIRGKVQKEYAFFYKLDIIPIDNDTTSYKLTSCAEAAAKEAAAKAPIPIHYCAPAGFAILKCNNKTFNGTGPCTNVSTVCTRPNNNTRKRIRIQRGPGRAFVTIAEAAAKEAAAKAFGNNKTIIFKQSSGGDAEAAAKEAAAKAAEAAAKEAAAKAPCRIKQIINMWQKVGKAMYAPPISGQIAEAAAKEAAAKALTRDGGNSNNESEIFRPGGGDAEAAAKEAAAKAIEPLGVAPTKAKRRVVQREKGGGPSGGGPSKPLDGEYFTLQIRGRERFEMFRELNEALELKDAQAGKEPGHHHHHHH

SEQ ID NO: 6 - protein, 405 aa, Synthetic
MYRMQLLSCIALSLALVTNSCTDLKNDTNTNSSSGRMIMEKTWIQNPGTKWYQNPGTKIYTTSIRGKVQKEYAFFYKLDIIPIDNDTTSYKLTSCTWIQNPGTKWYQNPGTKIYTPIPIHYCAPAGFAILKCNNKTFNGTGPCTNVSTVTWIQNPGTKWYQNPGTKIYTCTRPNNNTRKRIRIQRGPGRAFVTITWIQNPGTKWYQNPGTKIYTFGNNKTIIFKQSSGGDTWIQNPGTKWYQNPGTKIYTPCRIKQIINMWQKVGKAMYAPPISGQIAEAAAKEAAAKALTRDGGNSNNESEIFRPGGGDAEAAAKEAAAKAIEPLGVAPTKAKRRVVQREKRGGGPSNMWKNDMVEQMHEDIISLWGGGPSGYIPEAPRDGQAYVRKDGEWVLLSTFLHHHHHH

SEQ ID NO: 7 - protein, 477 aa, Synthetic
MYRMQLLSCIALSLALVTNSCTDLKNDTNTNSSSGRMIMEKTWIQNPGTKWYQNPGTKIYTTSIRGKVQKEYAFFYKLDIIPIDNDTTSYKLTSCTWIQNPGTKWYQNPGTKIYTPIPIHYCAPAGFAILKCNNKTFNGTGPCTNVSTVTWIQNPGTKWYQNPGTKIYTCTRPNNNTRKRIRIQRGPGRAFVTITWIQNPGTKWYQNPGTKIYTFGNNKTIIFKQSSGGDTWIQNPGTKWYQNPGTKIYTPCRIKQIINMWQKVGKAMYAPPISGQIAEAAAKEAAAKALTRDGGNSNNESEIFRPGGGDAEAAAKEAAAKAIEPLGVAPTKAKRRVVQREKRGGGPSNMWKNDMVEQMHEDIISLWGGGPSGGGPSGSHMWKQSVELAKKDSLYKDAMQYASESKDTELAEELLQWFLQEEKRECFGACLFTCYDLLRPDVVLELAWRHNIMDFAMPYFIQVMKEYLTKVHHHHHH

SEQ ID NO: 8 - protein, 526 aa, Synthetic
MYRMQLLSCIALSLALVTNSAVGIAVGIAEAAAKEAAAKAGALFLGFLGAAGSTMGAASMTLTVQARQLLSAEAAAKEAAAKAEAQQHLLQLTVWGIKQLQARILAVERYLKDQQLLGIWGCSGKLICTTAVPWNASWSAEAAAKEAAAKATSLIHSLIEESQNQQEKNEQELLELDKWASLWNWFNITNWLWYIKLFIAEAAAKEAAAKAPRGPDRPEGIEEEGGERDRDRSIAEAAAKEAAAKAYHRLRDLLLIVTRIVELLGRRGWEAEAAAKEAAAKAGTDRVIEVVQGACRAIRHIPRRIRQGLAPNLLGGPSVFIFPPKIKDVLMISLSPIVTCVVVDVSEDDPDVQISWFVNNVEVHTAQTQTHREDYNSTLRVVSALPIQHQDWMSGKEFKCKVNNKDLPAPIERTISKPKGSVRAPQVYVLPPPEEEMTKKQVTLTCMVTDFMPEDIYVEWTNNGKTELNYKNTEPVLDSDGSYFMYSKLRVEKKNWVERNSYSCSVVHEGLHNHHTTKSFSRTPGK

SEQ ID NO: 9 - protein, 523 aa, Synthetic
MYRMQLLSCIALSLALVTNSAVGIAVGIAEAAAKEAAAKAGALFLGFLGAAGSTMGAASMTLTVQARQLLSAEAAAKEAAAKAEAQQHLLQLTVWGIKQLQARILAVERYLKDQQLLGIWGCSGKLICTTAVPWNASWSAEAAAKEAAAKATSLIHSLIEESQNQQEKNEQELLELDKWASLWNWFNITNWLWYIKLFIAEAAAKEAAAKAPRGPDRPEGIEEEGGERDRDRSIAEAAAKEAAAKAYHRLRDLLLIVTRIVELLGRRGWEAEAAAKEAAAKAGTDRVIEVVQGACRAIRHIPRRIRQGLVPEVSSVFIFPPKPKDVLTITLTPKVTCVVVDISKDDPEVQFSWFVDDVEVHTAQTQPREEQFNSTFRSVSELPIMHQDWLNGKEFKCRVNSAAFPAPIEKTISKTKGRPKAPQVYTIPPPKEQMAKDKVSLTCMITDFFPEDITVEWQWNGQPAENYKNTQPIMDTDGSYFVYSKLNVQKSNWEAGNTFTCSVLHEGLHNHHTEKSLSHSPGI

SEQ ID NO: 10 - protein, 624 aa, Synthetic
MYRMQLLSCIALSLALVTNSAWEDADTTLFCASDAKAYSTEKHNVWATHACVPTDPDPQEIPLENVTENFNMWKNNMVEQMHEDIISLWDESLKPCVMLTGGSTIKQACPKVTFEPIPIHYCAPAGFAILKCRDEDFNGTGPCKNVSTVQCTHGIKPVVSTQLLLNGSLAKGDIVIRSENLTNNAKVIIVQLNEPVQIVCIRPNNGGSGSGGDIRQAHCNVTRSRWNKTLQEVKEQLWKIFNKTTNITFNNTIFNSPAGGDLEITTHSFNCGGEFFYCNTSDLFNETNLSANHTDTNENITLQCRIKQIVRMWQRVGQAMYAPPIAGNITCISNITGLLLTRDGVNDTHDKENETFRPTGGDMRDNWRSELYKYKVVRIEINFANSTGGDLEITTHSFNAPNLLGGPSVFIFPPKIKDVLMISLSPIVTCVVVDVSEDDPDVQISWFVNNVEVHTAQTQTHREDYNSTLRVVSALPIQHQDWMSGKEFKCKVNNKDLPAPIERTISKPKGSVRAPQVYVLPPPEEEMTKKQVTLTCMVTDFMPEDIYVEWTNNGKTELNYKNTEPVLDSDGSYFMYSKLRVEKKNWVERNSYSCSVVHEGLHNHHTTKSFSRTPGKHHHHHHHH

SEQ ID NO: 11 - protein, 639 aa, Synthetic
MYRMQLLSCIALSLALVTNSAWEDADTTLFCASDAKAYSTEKHNVWATHACVPTDPDPQEIPLENVTENFNMWKNNMVEQMHEDIISLWDESLKPCVMLTGGSTIKQACPKVTFEPIPIHYCAPAGFAILKCRDEDFNGTGPCKNVSTVQCTHGIKPVVSTQLLLNGSLAKGDIVIRSENLTNNAKVIIVQLNEPVQIVCIRPNNGGSGSGGDIRQAHCNVTRSRWNKTLQEVKEQLWKIFNKTTNITFNNTIFNSPAGGDLEITTHSFNCGGEFFYCNTSDLFNETNLSANHTDTNENITLQCRIKQIVRMWQRVGQAMYAPPIAGNITCISNITGLLLTRDGVNDTHDKENETFRPTGGDMRDNWRSELYKYKVVRIEINFANSTGGDLEITTHSFNPRGPTIKPCPPCKCPAPNLLGGPSVFIFPPKIKDVLMISLSPIVTCVVVDVSEDDPDVQISWFVNNVEVHTAQTQTHREDYNSTLRVVSALPIQHQDWMSGKEFKCKVNNKDLPAPIERTISKPKGSVRAPQVYVLPPPEEEMTKKQVTLTCMVTDFMPEDIYVEWTNNGKTELNYKNTEPVLDSDGSYFMYSKLRVEKKNWVERNSYSCSVVHEGLHNHHTTKSFSRTPGKHHHHHHHH

SEQ ID NO: 12 - protein, 611 aa, Synthetic
MYRMQLLSCIALSLALVTNSAWEDADTTLFCASDAKAYSTEKHNVWATHACVPTDPDPQEIPLENVTENFNMWKNNMVEQMHEDIISLWDESLKPCVMLTGGSTIKQACPKVTFEPIPIHYCAPAGFAILKCRDEDFNGTGPCKNVSTVQCTHGIKPVVSTQLLLNGSLAKGDIVIRSENLTNNAKVIIVQLNEPVQIVDIRQAHCNVTRSRWNKTLQEVKEQLWKIFNKTTNITFNNTIFNSPAGGDLEITTHSFNCGGEFFYCNTSDLFNETNLSANHTDTNENITLQCRIKQIVRMWQRVGQAMYAPPIAGNITCISNITGLLLTRDGVNDTHDKENETFRPTGGDMRDNWRSELYKYKVVRIEINFANSTGGDLEITTHSFNAPNLLGGPSVFIFPPKIKDVLMISLSPIVTCVVVDVSEDDPDVQISWFVNNVEVHTAQTQTHREDYNSTLRVVSALPIQHQDWMSGKEFKCKVNNKDLPAPIERTISKPKGSVRAPQVYVLPPPEEEMTKKQVTLTCMVTDFMPEDIYVEWTNNGKTELNYKNTEPVLDSDGSYFMYSKLRVEKKNWVERNSYSCSVVHEGLHNHHTTKSFSRTPGKHHHHHHHH

SEQ ID NO: 13 - protein, 626 aa, Synthetic
MYRMQLLSCIALSLALVTNSAWEDADTTLFCASDAKAYSTEKHNVWATHACVPTDPDPQEIPLENVTENFNMWKNNMVEQMHEDIISLWDESLKPCVMLTGGSTIKQACPKVTFEPIPIHYCAPAGFAILKCRDEDFNGTGPCKNVSTVQCTHGIKPVVSTQLLLNGSLAKGDIVIRSENLTNNAKVIIVQLNEPVQIVDIRQAHCNVTRSRWNKTLQEVKEQLWKIFNKTTNITFNNTIFNSPAGGDLEITTHSFNCGGEFFYCNTSDLFNETNLSANHTDTNENITLQCRIKQIVRMWQRVGQAMYAPPIAGNITCISNITGLLLTRDGVNDTHDKENETFRPTGGDMRDNWRSELYKYKVVRIEINFANSTGGDLEITTHSFNPRGPTIKPCPPCKCPAPNLLGGPSVFIFPPKIKDVLMISLSPIVTCVVVDVSEDDPDVQISWFVNNVEVHTAQTQTHREDYNSTLRVVSALPIQHQDWMSGKEFKCKVNNKDLPAPIERTISKPKGSVRAPQVYVLPPPEEEMTKKQVTLTCMVTDFMPEDIYVEWTNNGKTELNYKNTEPVLDSDGSYFMYSKLRVEKKNWVERNSYSCSVVHEGLHNHHTTKSFSRTPGKHHHHHHHH

SEQ ID NO: 14 - protein, 800 aa, Synthetic
MYRMQLLSCIALSLALVTNSAWEDADTTLFCASDAKAYSTEKHNVWATHACVPTDPDPQEIPLENVTENFNMWKNNMVEQMHEDIISLWDESLKPCVMLTGGSTIKQACPKVTFEPIPIHYCAPAGFAILKCRDEDFNGTGPCKNVSTVQCTHGIKPVVSTQLLLNGSLAKGDIVIRSENLTNNAKVIIVQLNEPVQIVCIRPNNGGSGSGGDIRQAHCNVTRSRWNKTLQEVKEQLWKIFNKTTNITFNNTIFNSPAGGDLEITTHSFNCGGEFFYCNTSDLFNETNLSANHTDTNENITLQCRIKQIVRMWQRVGQAMYAPPIAGNITCISNITGLLLTRDGVNDTHDKENETFRPTGGDMRDNWRSELYKYKVVRIEINFANSTGGDLEITTHSFNAPNLLGGPSVFIFPPKIKDVLMISLSPIVTCVVVDVSEDDPDVQISWFVNNVEVHTAQTQTHREDYNSTLRVVSALPIQHQDWMSGKEFKCKVNNKDLPAPIERTISKPKGSVRAPQVYVLPPPEEEMTKKQVTLTCMVTDFMPEDIYVEWTNNGKTELNYKNTEPVLDSDGSYFMYSKLRVEKKNWVERNSYSCSVVHEGLHNHHTTKSFSRTPGKAEAAAKEAAAKAAVGIGAVFLGFLGAAGSTMGAASMTLTVQARNLLSGIVQQQSNLLRAPEAQQHLLKLTVWGIKQLQARVLAVERYLRDQQLLGIWGCSGKLICCTNVPWNSSWSNRNLSEIWDNMTWLQWDKEISNYTQIIYGLLEESQNQQEKNEQDLLALDKWASLWNWFDITNWLWYIQ

SEQ ID NO: 15 - protein, 815 aa, Synthetic
MYRMQLLSCIALSLALVTNSAWEDADTTLFCASDAKAYSTEKHNVWATHACVPTDPDPQEIPLENVTENFNMWKNNMVEQMHEDIISLWDESLKPCVMLTGGSTIKQACPKVTFEPIPIHYCAPAGFAILKCRDEDFNGTGPCKNVSTVQCTHGIKPVVSTQLLLNGSLAKGDIVIRSENLTNNAKVIIVQLNEPVQIVCIRPNNGGSGSGGDIRQAHCNVTRSRWNKTLQEVKEQLWKIFNKTTNITFNNTIFNSPAGGDLEITTHSFNCGGEFFYCNTSDLFNETNLSANHTDTNENITLQCRIKQIVRMWQRVGQAMYAPPIAGNITCISNITGLLLTRDGVNDTHDKENETFRPTGGDMRDNWRSELYKYKVVRIEINFANSTGGDLEITTHSFNPRGPTIKPCPPCKCPAPNLLGGPSVFIFPPKIKDVLMISLSPIVTCVVVDVSEDDPDVQISWFVNNVEVHTAQTQTHREDYNSTLRVVSALPIQHQDWMSGKEFKCKVNNKDLPAPIERTISKPKGSVRAPQVYVLPPPEEEMTKKQVTLTCMVTDFMPEDIYVEWTNNGKTELNYKNTEPVLDSDGSYFMYSKLRVEKKNWVERNSYSCSVVHEGLHNHHTTKSFSRTPGKAEAAAKEAAAKAAVGIGAVFLGFLGAAGSTMGAASMTLTVQARNLLSGIVQQQSNLLRAPEAQQHLLKLTVWGIKQLQARVLAVERYLRDQQLLGIWGCSGKLICCTNVPWNSSWSNRNLSEIWDNMTWLQWDKEISNYTQIIYGLLEESQNQQEKNEQDLLALDKWASLWNWFDITNWLWYIQ

SEQ ID NO: 16 - protein, 787 aa, Synthetic
MYRMQLLSCIALSLALVTNSAWEDADTTLFCASDAKAYSTEKHNVWATHACVPTDPDPQEIPLENVTENFNMWKNNMVEQMHEDIISLWDESLKPCVMLTGGSTIKQACPKVTFEPIPIHYCAPAGFAILKCRDEDFNGTGPCKNVSTVQCTHGIKPVVSTQLLLNGSLAKGDIVIRSENLTNNAKVIIVQLNEPVQIVDIRQAHCNVTRSRWNKTLQEVKEQLWKIFNKTTNITFNNTIFNSPAGGDLEITTHSFNCGGEFFYCNTSDLFNETNLSANHTDTNENITLQCRIKQIVRMWQRVGQAMYAPPIAGNITCISNITGLLLTRDGVNDTHDKENETFRPTGGDMRDNWRSELYKYKVVRIEINFANSTGGDLEITTHSFNAPNLLGGPSVFIFPPKIKDVLMISLSPIVTCVVVDVSEDDPDVQISWFVNNVEVHTAQTQTHREDYNSTLRVVSALPIQHQDWMSGKEFKCKVNNKDLPAPIERTISKPKGSVRAPQVYVLPPPEEEMTKKQVTLTCMVTDFMPEDIYVEWTNNGKTELNYKNTEPVLDSDGSYFMYSKLRVEKKNWVERNSYSCSVVHEGLHNHHTTKSFSRTPGKAEAAAKEAAAKAAVGIGAVFLGFLGAAGSTMGAASMTLTVQARNLLSGIVQQQSNLLRAPEAQQHLLKLTVWGIKQLQARVLAVERYLRDQQLLGIWGCSGKLICCTNVPWNSSWSNRNLSEIWDNMTWLQWDKEISNYTQIIYGLLEESQNQQEKNEQDLLALDKWASLWNWFDITNWLWYIQ

SEQ ID NO: 17 - protein, 802 aa, Synthetic
MYRMQLLSCIALSLALVTNSAWEDADTTLFCASDAKAYSTEKHNVWATHACVPTDPDPQEIPLENVTENFNMWKNNMVEQMHEDIISLWDESLKPCVMLTGGSTIKQACPKVTFEPIPIHYCAPAGFAILKCRDEDFNGTGPCKNVSTVQCTHGIKPVVSTQLLLNGSLAKGDIVIRSENLTNNAKVIIVQLNEPVQIVDIRQAHCNVTRSRWNKTLQEVKEQLWKIFNKTTNITFNNTIFNSPAGGDLEITTHSFNCGGEFFYCNTSDLFNETNLSANHTDTNENITLQCRIKQIVRMWQRVGQAMYAPPIAGNITCISNITGLLLTRDGVNDTHDKENETFRPTGGDMRDNWRSELYKYKVVRIEINFANSTGGDLEITTHSFNPRGPTIKPCPPCKCPAPNLLGGPSVFIFPPKIKDVLMISLSPIVTCVVVDVSEDDPDVQISWFVNNVEVHTAQTQTHREDYNSTLRVVSALPIQHQDWMSGKEFKCKVNNKDLPAPIERTISKPKGSVRAPQVYVLPPPEEEMTKKQVTLTCMVTDFMPEDIYVEWTNNGKTELNYKNTEPVLDSDGSYFMYSKLRVEKKNWVERNSYSCSVVHEGLHNHHTTKSFSRTPGKAEAAAKEAAAKAAVGIGAVFLGFLGAAGSTMGAASMTLTVQARNLLSGIVQQQSNLLRAPEAQQHLLKLTVWGIKQLQARVLAVERYLRDQQLLGIWGCSGKLICCTNVPWNSSWSNRNLSEIWDNMTWLQWDKEISNYTQIIYGLLEESQNQQEKNEQDLLALDKWASLWNWFDITNWLWYIQ

SEQ ID NO: 18 - protein, 802 aa, Synthetic; identical to SEQ ID NO: 17

SEQ ID NO: 19 - protein, 436 aa, Synthetic
MYRMQLLSCIALSLALVTNSPRGPTIKPCPPCKCPAPNLLGGPSVFIFPPKIKDVLMISLSPIVTCVVVDVSEDDPDVQISWFVNNVEVHTAQTQTHREDYNSTLRVVSALPIQHQDWMSGKEFKCKVNNKDLPAPIERTISKPKGSVRAPQVYVLPPPEEEMTKKQVTLTCMVTDFMPEDIYVEWTNNGKTELNYKNTEPVLDSDGSYFMYSKLRVEKKNWVERNSYSCSVVHEGLHNHHTTKSFSRTPGKAEAAAKEAAAKAAVGIGAVFLGFLGAAGSTMGAASMTLTVQARNLLSGIVQQQSNLLRAPEAQQHLLKLTVWGIKQLQARVLAVERYLRDQQLLGIWGCSGKLICCTNVPWNSSWSNRNLSEIWDNMTWLQWDKEISNYTQIIYGLLEESQNQQEKNEQDLLALDKWASLWNWFDITNWLWYIQ

SEQ ID NO: 20 - protein, 522 aa, Synthetic
MYRMQLLSCIALSLALVTNSAVGIGALFLGFLGAAGSTMGAASMTLTVQARQLLSAEAAAKEAAAKAEAQQHLLQLTVWGIKQLQARILAVERYLKDQQLLGIWGCSGKLICTTAVPWNASWSAEAAAKEAAAKATSLIHSLIEESQNQQEKNEQELLELDKWASLWNWFNITNWLWYIKLFIAEAAAKEAAAKAPRGPDRPEGIEEEGGERDRDRSIAEAAAKEAAAKAYHRLRDLLLIVTRIVELLGRRGWEAEAAAKEAAAKAGTDRVIEVVQGACRAIRHIPRRIRQGLAEAAAKEAAAKAAPNLLGGPSVFIFPPKIKDVLMISLSPIVTCVVVDVSEDDPDVQISWFVNNVEVHTAQTQTHREDYNSTLRVVSALPIQHQDWMSGKEFKCKVNNKDLPAPIERTISKPKGSVRAPQVYVLPPPEEEMTKKQVTLTCMVTDFMPEDIYVEWTNNGKTELNYKNTEPVLDSDGSYFMYSKLRVEKKNWVERNSYSCSVVHEGLHNHHTTKSFSRTPGK

SEQ ID NO: 21 - protein, 835 aa, Synthetic
MYRMQLLSCIALSLALVTNSAVGIGALFLGFLGAAGSTMGAASMTLTVQARQLLSAEAAAKEAAAKAEAQQHLLQLTVWGIKQLQARILAVERYLKDQQLLGIWGCSGKLICTTAVPWNASWSAEAAAKEAAAKATSLIHSLIEESQNQQEKNEQELLELDKWASLWNWFNITNWLWYIKLFIAEAAAKEAAAKAPRGPDRPEGIEEEGGERDRDRSIAEAAAKEAAAKAYHRLRDLLLIVTRIVELLGRRGWEAEAAAKEAAAKAGTDRVIEVVQGACRAIRHIPRRIRQGLAEAAAKEAAAKAAPNLLGGPSVFIFPPKIKDVLMISLSPIVTCVVVDVSEDDPDVQISWFVNNVEVHTAQTQTHREDYNSTLRVVSALPIQHQDWMSGKEFKCKVNNKDLPAPIERTISKPKGSVRAPQVYVLPPPEEEMTKKQVTLTCMVTDFMPEDIYVEWTNNGKTELNYKNTEPVLDSDGSYFMYSKLRVEKKNWVERNSYSCSVVHEGLHNHHTTKSFSRTPGKAEAAAKEAAAKANMWKNDMVEQMHEDIISLWCTDLKNDTNTNSSSGRMIMEKAEAAAKEAAAKATSIRGKVQKEYAFFYKLDIIPIDNDTTSYKLTSCAEAAAKEAAAKAPIPIHYCAPAGFAILKCNNKTFNGTGPCTNVSTVCTRPNNNTRKRIRIQRGPGRAFVTIAEAAAKEAAAKAFGNNKTIIFKQSSGGDAEAAAKEAAAKAAEAAAKEAAAKAPCRIKQIINMWQKVGKAMYAPPISGQIAEAAAKEAAAKALTRDGGNSNNESEIFRPGGGDAEAAAKEAAAKAIEPLGVAPTKAKRRVVQREK

SEQ ID NO: 22 - protein, 714 aa, Synthetic
MYRMQLLSCIALSLALVTNSASMTLTVQARQLLSGIVQQQNNLLRAIEAQQHLLQLTVWGIKQLQARILAVERYLKDQQLLGIWGCSGKLICTTAVPWNASWSNKSLEQIWNHTTWMEWDREINNYTSLIHSLIEESQNQQEKNEQELLELDKWASLWNWFNITNWLWYIKLAEAAAKEAAAKAAPNLLGGPSVFIFPPKIKDVLMISLSPIVTCVVVDVSEDDPDVQISWFVNNVEVHTAQTQTHREDYNSTLRVVSALPIQHQDWMSGKEFKCKVNNKDLPAPIERTISKPKGSVRAPQVYVLPPPEEEMTKKQVTLTCMVTDFMPEDIYVEWTNNGKTELNYKNTEPVLDSDGSYFMYSKLRVEKKNWVERNSYSCSVVHEGLHNHHTTKSFSRTPGKAEAAAKEAAAKANMWKNDMVEQMHEDIISLWCTDLKNDTNTNSSSGRMIMEKAEAAAKEAAAKATSIRGKVQKEYAFFYKLDIIPIDNDTTSYKLTSCAEAAAKEAAAKAPIPIHYCAPAGFAILKCNNKTFNGTGPCTNVSTVCTRPNNNTRKRIRIQRGPGRAFVTIAEAAAKEAAAKAFGNNKTIIFKQSSGGDAEAAAKEAAAKAAEAAAKEAAAKAPCRIKQIINMWQKVGKAMYAPPISGQIAEAAAKEAAAKALTRDGGNSNNESEIFRPGGGDAEAAAKEAAAKAIEPLGVAPTKAKRRVVQREK

SEQ ID NO: 23 - protein, 416 aa, Synthetic
MYRMQLLSCIALSLALVTNSVFRPGGGDMRDNWRSELYKYKVIKIEPLGIAPTKAKRRVVQREKRQARQLLSGIVQQQNNLLRAIEAQQHLLQLTVWGIKQLQARVLAVERYLRDQQLLGIWGCSGKLICTTAVPWNASWSNKSLEDIWDNMTWMQWEREIDNYTNTIYTLLEESQNQQEKNEQELLGGGGSGGGGSGGGGSVPEVSSVFIFPPKPKDVLTITLTPKVTCVVVDISKDDPEVQFSWFVDDVEVHTAQTQPREEQFNSTFRSVSELPIMHQDWLNGKEFKCRVNSAAFPAPIEKTISKTKGRPKAPQVYTIPPPKEQMAKDKVSLTCMITDFFPEDITVEWQWNGQPAENYKNTQPIMDTDGSYFVYSKLNVQKSNWEAGNTFTCSVLHEGLHNHHTEKSLSHSPGK

SEQ ID NO: 24 - protein, 416 aa, Synthetic
MYRMQLLSCIALSLALVTNSVPEVSSVFIFPPKPKDVLTITLTPKVTCVVVDISKDDPEVQFSWFVDDVEVHTAQTQPREEQFNSTFRSVSELPIMHQDWLNGKEFKCRVNSAAFPAPIEKTISKTKGRPKAPQVYTIPPPKEQMAKDKVSLTCMITDFFPEDITVEWQWNGQPAENYKNTQPIMDTDGSYFVYSKLNVQKSNWEAGNTFTCSVLHEGLHNHHTEKSLSHSPGKGGGGSGGGGSGGGGSVFRPGGGDMRDNWRSELYKYKVIKIEPLGIAPTKAKRRVVQREKRQARQLLSGIVQQQNNLLRAIEAQQHLLQLTVWGIKQLQARVLAVERYLRDQQLLGIWGCSGKLICTTAVPWNASWSNKSLEDIWDNMTWMQWEREIDNYTNTIYTLLEESQNQQEKNEQELL

SEQ ID NO: 25 - protein, 416 aa, Synthetic
MYRMQLLSCIALSLALVTNSVPEVSSVFIFPPKPKDVLTITLTPKVTCVVVDISKDDPEVQFSWFVDDVEVHTAQTQPREEQFNSTFRSVSELPIMHQDWLNGKEFKCRVNSAAFPAPIEKTISKTKGRPKAPQVYTIPPPKEQMAKDKVSLTCMITDFFPEDITVEWQWNGQPAENYKNTQPIMDTDGSYFVYSKLNVQKSNWEAGNTFTCSVLHEGLHNHHTEKSLSHSPGKGGGGSGGGGSGGGGSIFRPGGGNMRDNWRSELYKYKVVKIEPLGVAPSRAKRRVVEREKRQARQLLSGIVQQQSNLLRAIEAQQHLLQLTVWGIKQLQARVLAVERYLKDQQLLGIWGCSGKLICTTNVPWNSSWSNKSMNEIWDNMTWLQWDKEISNYTQIIYNLIEESQNQQEKNEQDLL

SEQ ID NO: 26 - protein, 416 aa, Synthetic
MYRMQLLSCIALSLALVTNSVPEVSSVFIFPPKPKDVLTITLTPKVTCVVVDISKDDPEVQFSWFVDDVEVHTAQTQPREEQFNSTFRSVSELPIMHQDWLNGKEFKCRVNSAAFPAPIEKTISKTKGRPKAPQVYTIPPPKEQMAKDKVSLTCMITDFFPEDITVEWQWNGQPAENYKNTQPIMDTDGSYFVYSKLNVQKSNWEAGNTFTCSVLHEGLHNHHTEKSLSHSPGKGGGGSGGGGSGGGGSTFRPGGGNMKDNWRSELYKYKVVEIKPLGIAPTGAKRRVVEREKRQARQLLSGIVQQQSNLLRAIEAQQHMLQLTVWGIKQLQTRVLAIERYLKDQQLLGLWGCSGRLICTTAVPWNSSWSNKTSADIWDNMTWMQWDREISNYTDTIYRLLEDSQNQQEKNEKDLL

SEQ ID NO: 27 - protein, 416 aa, Synthetic
MYRMQLLSCIALSLALVTNSVPEVSSVFIFPPKPKDVLTITLTPKVTCVVVDISKDDPEVQFSWFVDDVEVHTAQTQPREEQFNSTFRSVSELPIMHQDWLNGKEFKCRVNSAAFPAPIEKTISKTKGRPKAPQVYTIPPPKEQMAKDKVSLTCMITDFFPEDITVEWQWNGQPAENYKNTQPIMDTDGSYFVYSKLNVQKSNWEAGNTFTCSVLHEGLHNHHTEKSLSHSPGKGGGGSGGGGSGGGGSVFRPGGGNMRDNWRSELYKYKVVKIEPLGVAPTKAKRRVVEREKRQARQLLSGIVQQQSNLLRAIEAQQHLLQLTVWGIKQLQARVLAVERYLKDQQLLGIWGCSGKLICTTAVPWNSSWSNKSLNKIWDNMTWMEWDREISNYTSIIYSLIEESQNQQEKNEQDLL

SEQ ID NO: 28 - protein, 425 aa, Synthetic
MYRMQLLSCIALSLALVTNSTNITFSAEVAELYRLELGDYKLVEVTPIGFAPTAEKRYSSAPGRHKRGVLVLQSRTLLAGIVQQQQQLLDVVKRQQEMLRLTVWGTKNLQARVTAIEKYLADQARLNSWGCAFRQVCHTTVPWVNDTLTPEWNNMTWQEWEHKIRFLEANISESLEQAQIQQEKNMYELQKLNSWDGGGGSGGGGSGGGGSVPEVSSVFIFPPKPKDVLTITLTPKVTCVVVDISKDDPEVQFSWFVDDVEVHTAQTQPREEQFNSTFRSVSELPIMHQDWLNGKEFKCRVNSAAFPAPIEKTISKTKGRPKAPQVYTIPPPKEQMAKDKVSLTCMITDFFPEDITVEWQWNGQPAENYKNTQPIMDTDGSYFVYSKLNVQKSNWEAGNTFTCSVLHEGLHNHHTEKSLSHSPGK

SEQ ID NO: 29 - protein, 425 aa, Synthetic
MYRMQLLSCIALSLALVTNSVPEVSSVFIFPPKPKDVLTITLTPKVTCVVVDISKDDPEVQFSWFVDDVEVHTAQTQPREEQFNSTFRSVSELPIMHQDWLNGKEFKCRVNSAAFPAPIEKTISKTKGRPKAPQVYTIPPPKEQMAKDKVSLTCMITDFFPEDITVEWQWNGQPAENYKNTQPIMDTDGSYFVYSKLNVQKSNWEAGNTFTCSVLHEGLHNHHTEKSLSHSPGKGGGGSGGGGSGGGGSTNITFSAEVAELYRLELGDYKLVEVTPIGFAPTAEKRYSSAPGRHKRGVLVLQSRTLLAGIVQQQQQLLDVVKRQQEMLRLTVWGTKNLQARVTAIEKYLADQARLNSWGCAFRQVCHTTVPWVNDTLTPEWNNMTWQEWEHKIRFLEANISESLEQAQIQQEKNMYELQKLNSWD

SEQ ID NO: 30 - protein, 467 aa, Synthetic
MYRMQLLSCIALSLALVTNSTHTLLKGIVQQQDNLLRAIQAQQQLLRLSVWGIRQLRARLLALETLLQNQQLLSLWGCKGKLVCYTSVKWNRTWIGNESIWDTLTWQEWDRQISNISSTIYEEIQKAQVQQEQNEKKLLELDEWASIWNWLDITKWLWYIKIAIIIVGALVGVRVIMIVLNIVKNIRQGYQPLSLQIPNHHQEEAGTPGRTGGGGGEEGRPRWIPSPQGFLPLLYTDLGGGGSGGGGSGGGGSVPEVSSVFIFPPKPKDVLTITLTPKVTCVVVDISKDDPEVQFSWFVDDVEVHTAQTQPREEQFNSTFRSVSELPIMHQDWLNGKEFKCRVNSAAFPAPIEKTISKTKGRPKAPQVYTIPPPKEQMAKDKVSLTCMITDFFPEDITVEWQWNGQPAENYKNTQPIMDTDGSYFVYSKLNVQKSNWEAGNTFTCSVLHEGLHNHHTEKSLSHSPGK

SEQ ID NO: 31 - protein, 467 aa, Synthetic
MYRMQLLSCIALSLALVTNSVPEVSSVFIFPPKPKDVLTITLTPKVTCVVVDISKDDPEVQFSWFVDDVEVHTAQTQPREEQFNSTFRSVSELPIMHQDWLNGKEFKCRVNSAAFPAPIEKTISKTKGRPKAPQVYTIPPPKEQMAKDKVSLTCMITDFFPEDITVEWQWNGQPAENYKNTQPIMDTDGSYFVYSKLNVQKSNWEAGNTFTCSVLHEGLHNHHTEKSLSHSPGKGGGGSGGGGSGGGGSTHTLLKGIVQQQDNLLRAIQAQQQLLRLSVWGIRQLRARLLALETLLQNQQLLSLWGCKGKLVCYTSVKWNRTWIGNESIWDTLTWQEWDRQISNISSTIYEEIQKAQVQQEQNEKKLLELDEWASIWNWLDITKWLWYIKIAIIIVGALVGVRVIMIVLNIVKNIRQGYQPLSLQIPNHHQEEAGTPGRTGGGGGEEGRPRWIPSPQGFLPLLYTDL

SEQ ID NO: 32 - protein, 401 aa, Synthetic
MYRMQLLSCIALSLALVTNSVPEVSSVFIFPPKPKDVLTITLTPKVTCVVVDISKDDPEVQFSWFVDDVEVHTAQTQPREEQFNSTFRSVSELPIMHQDWLNGKEFKCRVNSAAFPAPIEKTISKTKGRPKAPQVYTIPPPKEQMAKDKVSLTCMITDFFPEDITVEWQWNGQPAENYKNTQPIMDTDGSYFVYSKLNVQKSNWEAGNTFTCSVLHEGLHNHHTEKSLSHSPGKGGGGSGGGGSGGGGSASMTLTVQARQLLSGIVQQQNNLLRAIEAQQHLLQLTVWGIKQLQARILAVERYLKDQQLLGIWGCSGKLICTTAVPWNASWSNKSLEQIWNHTTWMEWDREINNYTSLIHSLIEESQNQQEKNEQELLELDKWASLWNWFNITNWLWYIKL

SEQ ID NO: 33 - protein, 401 aa, Synthetic
MYRMQLLSCIALSLALVTNSASMTLTVQARQLLSGIVQQQNNLLRAIEAQQHLLQLTVWGIKQLQARILAVERYLKDQQLLGIWGCSGKLICTTAVPWNASWSNKSLEQIWNHTTWMEWDREINNYTSLIHSLIEESQNQQEKNEQELLELDKWASLWNWFNITNWLWYIKLGGGGSGGGGSGGGGSVPEVSSVFIFPPKPKDVLTITLTPKVTCVVVDISKDDPEVQFSWFVDDVEVHTAQTQPREEQFNSTFRSVSELPIMHQDWLNGKEFKCRVNSAAFPAPIEKTISKTKGRPKAPQVYTIPPPKEQMAKDKVSLTCMITDFFPEDITVEWQWNGQPAENYKNTQPIMDTDGSYFVYSKLNVQKSNWEAGNTFTCSVLHEGLHNHHTEKSLSHSPGK

SEQ ID NO: 34 - protein, 865 aa, Synthetic
MYRMQLLSCIALSLALVTNSMRVKEKYQHLWRWGWKWGTMLLGILMICSATEKLWVTVYYGVPVWKEATTTLFCASDAKAYDTEVHNVWATHACVPTDPNPQEVVLVNVTENFNMWKNDMVEQMHEDIISLWDQSLKPCVKLTPLCVSLKCTDLGNATNTNSSNTNSSSGEMMMEKGEIKNCSFNISTSIRGKVQKEYAFFYKLDIIPIDNDTTSYTLTSCNTSVITQACPKVSFEPIPIHYCAPAGFAILKCNNKTFNGTGPCTNVSTVQCTHGIRPVVSTQLLLNGSLAEEEVVIRSANFTDNAKTIIVQLNQSVEINCTRPNNNTRKSIRIQRGPGRAFVTIGKIGNMRQAHCNISRAKWNATLKQIASKLREQFGNNKTIIFKQSSGGDPEIVTHSFNCGGEFFYCNSTQLFNSTWFNSTWSTEGSNNTEGSDTITLPCRIKQFINMWQEVGKAMYAPPISGQIRCSSNITGLLLTRDGGNNNNGSEIFRPGGGDMRDNWRSELYKYKVVKIEPLGVAPTKAQNHVVQNEHQAVGIGALFLGFLGAAGSTMGARSMTLTVQARQLLSGIVQQQNNLLRAIEAQQHLLQLTVWGIKQLQARILAVERYLKDQQLLGIWGCSGKLICTTAVPWNASWSNKSLEQIWNNMTWMEWDREINNYTSLIHSLIEESQNQQEKNEQELLELDKWASLWNWFNITNWLWYIKNRVRQGYSPLSFQTHLPTPRGPDRPEGIEEEGGERDRDRSIRLVNGSLALIWDDLRSLCLFSYHRLRDLLLIVTRIVELLGRRGWEALKYWWNLLQYWSQELKNSAVSLLNATAIAVAEGTDRVIEVVQGACRAIRHIPRRIRQGLERILLHHHHHH

SEQ ID NO: 35 - protein, 849 aa, Synthetic
MYRMQLLSCIALSLALVTNSMRVRGIQRNWPQWWIWGILGFWMVMICRVVVGNMWVTVYYGVPVWKEAKTTLFCASDAKAYEKEVHNVWATHACVPTDPNPQEIVLENVTENFNMWKNDMVDQMHEDIISLWDQSLKPCVKLAPLCVTLNCTNSNATYNNSMHGEIKNCSFNTTTEIRDKKQNVYALFYKSDVVPLKEDNDNSSYSSYILINCNTSTITQACPKVTFDPIPIHYCAPAGYAILKCNNKTFNGTGPCSNVSTVQCTHGIKPVVSTQLLLNGSLAEGEIIIRSENLTNNIKTIIVQLNTSREIVCTRPNNNTRKSIRIGPGQAFYATNEIIGDIRQAYCNISKTEWSTTLDEVKKKLAEHFPNKTIRFAPPIGGDLEITTHSFNCRGEFFYCNTTELFNDNNSDDNATITLPCRIKQIINMWQGVGRAMYAPPIEGSITCNSNITGLLLTRDGGTNNTDETFRPGGGNMKDNWRSELYKYKVVEIKPLGIAPTKAQNHVVQNEHQAVGLGAVFLGFLGAAGSTMGAASITLTVQARQLLSGIVQQQSNLLRAIEAQQHMLQLTVWGIKQLQTRVLAIERYLKDQQLLGLWGCSGRLICTTAVPWNSSWSNKTSADIWDNMTWMQWDREISNYTDTIYRLLEDSQNQQEKNEKDLLALDSWKNLWNWFNITNWLWYIKKRVRQGYSPLSFQTLTPNPRELDRLGRIEEEGGEQDKDRSIRLVNGFLSLAWDDLRSLCLFSYHQLRDFILIVARVVELLGRSSLRGLQRGWEALKYLGNLVQYWGLELKKSAISLFDNIAITVAERTDRILELIYRIYRAIRNIPRRIRQGFEVALLHHHHHH

SEQ ID NO: 36 - protein, 850 aa, Synthetic
MYRMQLLSCIALSLALVTNSMRVRGIQTSWQNLWRWGTMILGMLMIYSAAENLWVTVYYGVPVWKDAETTLFCASDAKAYDTEVHNVWATHACVPTDPNPQEIHLENVTEDFNMWKNNMVEQMHTDIISLWDQSLKPCVKLTPLCVTLDCNATASNVTNEMRNCSFNITTELKDKKQQVYSLFYKLDVVQINEKNETDKYRLINCNTSAITQACPKVSFEPIPIHYCAPAGFAILKCKDTEFNGTGPCKNVSTVQCTHGIRPVISTQLLLNGSLAEEGIQIRSENITNNAKTIIVQLDKAVKINCTRPNNNTRKGVRIGPGQAFYATGGIIGDIRQAHCNVSRAKWNDTLRGVAKKLREHFKNKTIIFEKSSGGDIEITTHSFNCGGEFFYCNTSGLFNSTWESNSTESNNTTSNDTITLTCRIKQIINMWQKVGQAMYAPPIQGVIRCESNITGLLLTRDGGNNSTNEIFRPGGGNMRDNWRSELYKYKVVKIEPLGVAPSKAQNHVVQNEHQAVGIGAVFLGFLGAAGSTMGAASITLTAQARQLLSGIVQQQSNLLRAIEAQQHMLKLTVWGIKQLQARVLAVERYLKDQQLLGIWGCSGKLICTTNVPWNSSWSNKSMNEIWDNMTWLQWDKEISNYTQIIYNLIEESQNQQEKNEQDLLALDKWASLWNWFDISRWLWYIKNRVRQGYSPLSFQIRTPNPKEPDRLGRIDGEGGEQDRDRSIRLVSGFLALAWDDLRSLCLFSYHRLRDFISIAARTVELLGHSSLKGLRLGWEGLKYLWNLLLYWGRELKTSAVNLVDTIAIAVAGWTDRVIEVGQRIFRAILNIPRRIRQGLERGLLHHHHHH

SEQ ID NO: 37 - protein, 868 aa, Synthetic
MYRMQLLSCIALSLALVTNSVKETQMNWPNLWKWGTLILGLVIICSAADNLWVTVYYGVPVWRDADTTLFCASDAKAHETEVHNVWATHACVPTDPNPQEIHLENVTENFNMWKNNMVEQMQEDVISLWDQSLKPCVKLTPFCVTLNCTNATLTNVTNIANASNMIGNITDEIRNCSFNMTTELRDKKQQVHALFYKLDIVQIEDNKNSSNNSSNSSKYSEYRLINCNTSVIKQACPKISFDPIPIHYCTPAGYAILKCNDKNFNGTGPCKNVSSVQCTHGIKPVVSTQLLLNGSLAEEEIIIRSENLTNNAKTIIVHLNKSVEINCTRPFYTRISMTRGPGHVFYRTGKIVGDPRKAYCEINGTKWNEALKQVTEKLKEHFNKTIIFQPPSGGDLEITMHHFNCRGEFFYCNTTKLFNSTGIGNETMKGYNDTITLPCRIKQIINMWQGAGQAMYAPPIKERINCVSNITGILLTRDGGINSTTNETFRPGGGNIKDNWRSELYKYKVVQIEPLGIAPTKAQNHVVQNEHQAVGIGAVIFGFLGAAGSTMGAASITLTVQARQLLSGIVQQQSNLLRAIEAQQHLLQLTVWGIKQLQARVLAVERYLKDQQFLGLWGCSGKIICTTAVPWNSTWSNRSYEEIWNNMTWIEWEREISNYTNQIYEILTESQDQQDRNEKDLLELDKWASLWNWFNITNWLWYIKNRVRQGYSPLSFQIPSHHQREPDRPEGIEEGGGEEGRDRSVRLVSGFLALAWDDLRSLCLFSYHRLRDLLSIATRTVELLGHSSLKGLRRGWEGLKYLGNLLLYWGQELKISAISLLDTTAIAVAGWTDRVIEVAQRAWRAILHIPRRIRQGLERSLLHHHHHH

SEQ ID NO: 38 - protein, 879 aa, Synthetic
MYRMQLLSCIALSLALVTNSMRVKEKYQHLWKWGWRWGTMLLGMLMICNVAEENLWVTVYYGVPVWKEATTTLFCASDAKAYDTEVHNVWATHACVPTDPNPQEIELENVTENFNMWKNNMVEQMHEDIISLWDQSLKPCVKLTPLCVTLNCTDLRNATNGNDTNTTSSSREMMGGGEMKNCSFNITTEIRDKKQKVYALFYKLDIVPIDNNKNSSNNSSNSSSNNRYRLINCNTSVITQACPKISFEPIPIHYCAPAGFAILKCKDKKFNGTGPCSNVSTVQCTHGIRPVVSTQLLLNGSLAEEEIVIRSENFTNNAKTIIVQLNESVEINCTRPNNNTRKSIHIGPGRAFYTTGEIIGDIRQAHCNLSRAKWNDTLNKVVIKLREHFGNKTIVFKHSSGGDPEITTHSFNCGGEFFYCNTTQLFNSTWESNSTESNNTVENNTITLPCRIKQIINMWQKVGRAMYAPPIRGQIRCSSNITGLLLTRDGGPNANTTEVFRPGGGNMRDNWRSELYKYKVVKIEPLGVAPTKAQNHVVQNEHQAVGIGAVFLGFLGAAGSTMGAASITLTVQARQLLSGIVQQQSNLLRAIEAQQHLLQLTVWGIKQLQARVLAVERYLKDQQLLGIWGCSGKLICTTAVPWNSSWSNKSLNKIWDNMTWMEWDREISNYTSIIYSLIEESQNQQEKNEQDLLELDKWASLWNWFDITEWLWYIKNRVRQGYSPLSFQTHLPASREPDRPGGIEEEGGERDRDRSGRLVNGFLALAWDDLRSLCLFSYHRLRDLLLIVTRIVELLGRSSLRGLQRGWEFLKYLWNLLQYWGQELKNSAVSLLDTIAIAVAEGTDRVIEVLQRAVRAILHIPRRIRQGLERALLHHHHHH

SEQ ID NO: 39 - protein, 829 aa, Human immunodeficiency virus
MRVMGIQRNCQHLWRWGILIFGMLIICSAAENLWVTVYYGVPVWKEANTTLFCASDAKAYDTEVHNVWATHACVPTDPNPQEIVLENVTENFNMWKNNMVEQMHEDIISLWDQSLKPCVKLTPLCVTLNCTDVNATNNTTNNEEIKNCSFNITTEIRDKKKKVYALFYKLDVVPIDDNNSYRLINCNTSAITQACPKVSFEPIPIHYCAPAGFAILKCNDKKFNGTGPCKNVSTVQCTHGIKPVVSTQLLLNGSLAEEEIIIRSENITNNAKTIIVQLNESVEINCTRPNNNTRKSIRIGPGQAFYATGDIIGDIRQAHCNISRTKWNKTLQQVAKKLREHFNKTIIFNPSSGGDLEITTHSFNCGGEFFYCNTSELFNSTWNGTNNTITLPCRIKQIINMWQGVGQAMYAPPIEGKIRCTSNITGLLLTRDGGNNNTETFRPGGGDMRDNWRSELYKYKVVKIEPLGVAPTKAKRRVVEREKRAVGIGAVFLGFLGAAGSTMGAASITLTVQARQLLSGIVQQQSNLLRAIEAQQHLLQLTVWGIKQLQARVLAVERYLKDQQLLGIWGCSGKLICTTNVPWNSSWSNKSQDEIWDNMTWMEWDKEINNYTDIIYSLIEESQNQQEKNEQELLALDKWASLWNWFDITNWLWYIKIFIMIVGGLIGLRIVFAVLSIVNRVRQGYSPLSFQTLIPNPRGPDRPEGIEEEGGEQDRDRSIRLVNGFLALAWDDLRSLCLFSYHRLRDLILIAARTVELLGRRGWEALKYLWNLLQYWGQELKNSAISLLDTTAIAVAEGTDRVIEVVQRVCRAILNIPRRIRQGFERALL

SEQ ID NO: 40 - protein, 830 aa, Human immunodeficiency virus
MRVMGIQRNCQHLWRWGILIFGMLMICSAAENLWVTVYYGVPVWKEANTTLFCASDAKAYDTEVHNVWATHACVPTDPNPQEIVLENVTENFNMWKNNMVEQMHEDIISLWDQSLKPCVKLTPLCVTLNCTDVNATNNSTNMGEIKNCSFNITTEIRDKKQKVYALFYRLDVVPINDNNSYRLINCNTSAITQACPKVSFEPIPIHYCAPAGFAILKCNDKKFNGTGPCKNVSTVQCTHGIKPVVSTQLLLNGSLAEEEIIIRSENITDNAKTIIVQLNESVEINCTRPNNNTRKSIRIGPGQAFYATGDIIGDIRQAHCNISGAEWNKTLQQVAAKLREHFNNKTIIFKPSSGGDLEITTHSFNCGGEFFYCNTSGLFNSTWNGTNETITLPCRIKQIVNMWQRVGQAMYAPPIAGNITCKSNITGLLLTRDGGTNNTETFRPGGGDMRDNWRSELYKYKVVKIEPLGVAPTKAKRRVVEREKRAVGIGAVFLGFLGAAGSTMGAASITLTVQARQLLSGIVQQQSNLLRAIEAQQHLLQLTVWGIKQLQARVLAVERYLKDQQLLGIWGCSGKLICTTNVPWNSSWSNKSQDEIWDNMTWMQWEREISNYTDIIYSLIEESQNQQEKNEQDLLALDKWASLWNWFDITNWLWYIKIFIMIVGGLIGLRIVFAVLSIVNRVRQGYSPLSFQTLIPNPRGPDRPGGIEEEGGEQDRDRSIRLVSGFLALAWDDLRSLCLFSYHRLRDFILIAARTVELLGRRGWEALKYLWNLLQYWGQELKNSAISLLDTTAIAVAEGTDRVIEVVQRACRAILHIPRRIRQGFERALL

SEQ ID NO: 41 - protein, 845 aa, Human immunodeficiency virus
MRVMGIQRNCQHLLRWGTMILGMIIICSAAENLWVTVYYGVPVWKDAETTLFCASDAKAYETEMHNVWATHACVPTDPNPQEIHLENVTEEFNMWKNNMVEQMHTDIISLWDQSLKPCVKLTPLCVTLNCSNVNVTNNTTNTHEEEIKNCSFNMTTELRDKKQKVYSLFYRLDVVQINENNSNSSYRLINCNTSAITQACPKVSFEPIPIHYCAPAGFAILKCKDKEFNGTGPCKNVSTVQCTHGIKPVVSTQLLLNGSLAEEEVIIRSENITNNAKTIIVQLTKPVKINCTRPNNNTRKSIRIGPGQAFYATGDIIGDIRQAHCNVSRSEWNKTLQKVAKQLRKYFKNKTIIFTNSSGGDLEITTHSFNCGGEFFYCNTSGLFNSTWNNGTMKNTITLPCRIKQIINMWQRAGQAMYAPPIQGVIRCESNITGLLLTRDGGNNNTNETFRPGGGDMRDNWRSELYKYKVVKIEPLGVAPTRAKRRVVEREKRAVGIGAVFLGFLGAAGSTMGAASITLTVQARQLLSGIVQQQSNLLRAIEAQQHLLKLTVWGIKQLQARVLAVERYLKDQQLLGIWGCSGKLICTTNVPWNSSWSNKSQNEIWDNMTWLQWDKEISNYTHIIYNLIEESQNQQEKNEQDLLALDKWANLWNWFDISNWLWYIKIFIMIVGGLIGLRIVFAVLSVINRVRQGYSPLSFQTHTPNPRGLDRPGRIEEEGGEQGRDRSIRLVSGFLALAWDDLRSLCLFSYHRLRDFILIAARTVELLGHSSLKGLRLGWEGLKYLWNLLLYWGRELKISAINLVDTIAIAVAGWTDRVIEIGQRIGRAILHIPRRIRQGLERALL

SEQ ID NO: 42 - protein, 845 aa, Human immunodeficiency virus
MRVMGIQRNCQHLWRWGTMIFGMIIICSAAENLWVTVYYGVPVWKDAETTLFCASDAKAYDTEVHNVWATHACVPTDPNPQEIDLENVTEEFNMWKNNMVEQMHADIISLWDQSLKPCVKLTPLCVTLNCSNVNVTNNTTNTHEEEIKNCSFNMTTELRDKKQKVYSLFYRLDVVPINENNSNSSYRLINCNTSAITQACPKVSFEPIPIHYCAPAGFAILKCKDKEFNGTGPCKNVSTVQCTHGIKPVVSTQLLLNGSLAEEEVMIRSENITDNAKTIIVQLTEPVKINCTRPNNNTRKSIRIGPGQAFYATGDIIGDIRQAHCNVSRTEWNKTLQKVAAQLRKHFNNKTIIFNSSSGGDLEITTHSFNCGGEFFYCNTSGLFNSTWNNGTMKDTITLPCRIKQIINMWQRVGQAMYAPPIQGVIRCESNITGLLLTRDGGNNNTNETFRPGGGDMRDNWRSELYKYKVVKIEPLGVAPTRAKRRVVEREKRAVGLGAVFLGFLGAAGSTMGAASITLTVQARQLLSGIVQQQSNLLRAIEAQQHLLKLTVWGIKQLQARVLAVERYLKDQQLLGIWGCSGKLICTTNVPWNSSWSNKSQDEIWDNMTWLQWDKEISNYTDIIYNLIEESQNQQEKNEQDLLALDKWANLWNWFDISNWLWYIKIFIMIVGGLIGLRIVFAVLSVINRVRQGYSPLSFQTLTPNPEGPDRPGRIEEEGGEQGRDRSIRLVSGFLALAWDDLRSLCLFSYHRLRDFILIAARTVELLGRSSLKGLRLGWEGLKYLWNLLLYWGRELKISAINLLDTIAIAVAGWTDRVIEIGQRICRAILNIPRRIRQGLERALL

SEQ ID NO: 43 - protein, 843 aa, Human immunodeficiency virus
MRVMGTQRNYQHLWRWGILILGMLIMCKATDLWVTVYYGVPVWKDADTTLFCASDAKAYDTEVHNVWATHACVPTDPNPQEVNLENVTEDFNMWKNNMVEQMHEDIISLWDQSLKPCVKLTPLCVTLNCSNANTTNNSTMEEIKNCSYNITTELRDKTQKVYSLFYKLDVVQLDESNKSEYYYRLINCNTSAITQACPKVSFEPIPIHYCAPAGFAILKCKDPRFNGTGSCNNVSSVQCTHGIKPVASTQLLLNGSLAEGKVMIRSENITNNAKNIIVQFNKPVPITCIRPNNNTRKSIRFGPGQAFYTNDIIGDIRQAHCNINKTKWNATLQKVAEQLREHFPNKTIIFTNSSGGDLEITTHSFNCGGEFFYCNTTGLFNSTWKNGTTNNTEQMITLPCRIKQIINMWQRVGRAMYAPPIAGVIKCTSNITGIILTRDGGNNETETFRPGGGDMRDNWRSELYKYKVVKIEPLGVAPTRAKRRVVEREKRAVGMGAVFLGFLGAAGSTMGAASITLTVQARQLLSGIVQQQSNLLKAIEAQQHLLKLTVWGIKQLQARVLALERYLQDQQLLGIWGCSGKLICATTVPWNSSWSNKTQEEIWNNMTWLQWDKEISNYTNIIYKLLEESQNQQEKNEQDLLALDKWANLWNWFNITNWLWYIRIFIMIVGGLIGLRIVIAIISVVNRVRQGYSPLSFQIPTPNPEGLDRPGRIEEGGGEQGRDRSIRLVSGFLALAWDDLRSLCLFSYHRLRDCILIAARTVELLGHSSLKGLRLGWEGLKYLWNLLLYWGRELKNSAISLLDTIAVAVAEWTDRVIEIGQRACRAILNIPRRIRQGFERALL

SEQ ID NO: 44 - protein, 841 aa, Human immunodeficiency virus
MRVKGIRKNYQHLWRWGTMLLGMLMICSAAEKLWVTVYYGVPVWKEATTTLFCASDAKAYDTEVHNVWATHACVPTDPNPQEVVLENVTENFNMWKNNMVEQMHEDIISLWDQSLKPCVKLTPLCVTLNCTDLMNATNTNTTIIYRWRGEIKNCSFNITTSIRDKVQKEYALFYKLDVVPIDNDNTSYRLISCNTSVITQACPKVSFEPIPIHYCAPAGFAILKCNDKKFNGTGPCTNVSTVQCTHGIRPVVSTQLLLNGSLAEEEVVIRSENFTDNAKTIIVQLNESVEINCTRPNNNTRKSIHIGPGRAFYTTGEIIGDIRQAHCNISRAKWNNTLKQIVKKLREQFGNKTIVFNQSSGGDPEIVMHSFNCGGEFFYCNTTQLFNSTWNGTWNNTEGNITLPCRIKQIINMWQEVGKAMYAPPIRGQIRCSSNITGLLLTRDGGNNETEIFRPGGGDMRDNWRSELYKYKVVKIEPLGVAPTKAKRRVVQREKRAVGIGAMFLGFLGAAGSTMGAASMTLTVQARQLLSGIVQQQNNLLRAIEAQQHLLQLTVWGIKQLQARVLAVERYLKDQQLLGIWGCSGKLICTTAVPWNASWSNKSLDEIWDNMTWMEWEREIDNYTSLIYTLIEESQNQQEKNEQELLELDKWASLWNWFDITNWLWYIKIFIMIVGGLVGLRIVFAVLSIVNRVRQGYSPLSFQTRLPAPRGPDRPEGIEEEGGERDRDRSGRLVDGFLALIWDDLRSLCLFSYHRLRDLLLIVTRIVELLGRRGWEVLKYWWNLLQYWSQELKNSAVSLLNATAIAVAEGTDRVIEVVQRACRAILHIPRRIRQGLERALL

SEQ ID NO: 45 - protein, 840 aa, Human immunodeficiency virus
MRVKGIRKNCQHLWRWGTMLLGMLMICSAAENLWVTVYYGVPVWKEATTTLFCASDAKAYETEVHNVWATHACVPTDPNPQEVVLENVTENFNMWKNNMVEQMHEDIISLWDQSLKPCVKLTPLCVTLNCTDLLNATNTNSTNMYRWRGEIKNCSFNITTSIRDKMQKEYALFYKLDVVPIDNNTSYRLINCNTSVITQACPKVSFEPIPIHYCTPAGFAILKCNDKKFNGTGPCKNVSTVQCTHGIRPVVSTQLLLNGSLAEEEVVIRSENFTDNAKTIIVQLNESVEINCTRPNNNTRKSIHIGPGRAFYATGEIIGDIRQAHCNLSRAKWNNTLKQVVTKLREQFDNKTIVFNPSSGGDPEIVMHSFNCGGEFFYCNTTQLFNSTWNGTWNNTEGNITLPCRIKQIINMWQEVGKAMYAPPIRGQIRCSSNITGLLLTRDGGNNETEIFRPGGGDMRDNWRSELYKYKVVKIEPLGVAPTKAKRRVVQREKRAVGIGAMFLGFLGAAGSTMGAASMTLTVQARQLLSGIVQQQNNLLRAIEAQQHLLQLTVWGIKQLQARVLAVERYLRDQQLLGIWGCSGKLICTTTVPWNASWSNKSLDEIWNNMTWMEWEREIDNYTGLIYTLIEESQNQQEKNEQELLELDKWASLWNWFDITNWLWYIKIFIMIVGGLVGLRIVFAVLSIVNRVRQGYSPLSFQTRLPAPRGPDRPEGIEEEGGERDRDRSGRLVNGFLALIWDDLRSLCLFSYHRLRDLLLIVARIVELLGRRGWEALKYWWNLLQYWSQELKNSAVSLLNATAIAVAEGTDRVIEVVQRACRAILHIPRRIRQGLERALL

SEQ ID NO: 46 - protein, 835 aa, Human immunodeficiency virus
MRVRGILRNCQQWWIWGILGFWMLMICNVVGNLWVTVYYGVPVWKEAKTTLFCASDAKAYEKEVHNVWATHACVPTDPNPQEIVLENVTENFNMWKNDMVDQMHEDIISLWDQSLKPCVKLTPLCVTLNCTNATNATNTMGEIKNCSFNITTELRDKKQKVYALFYRLDIVPLNENNSYRLINCNTSAITQACPKVSFDPIPIHYCAPAGYAILKCNNKTFNGTGPCNNVSTVQCTHGIKPVVSTQLLLNGSLAEEEIIIRSENLTNNAKTIIVHLNESVEIVCTRPNNNTRKSIRIGPGQTFYATGDIIGDIRQAHCNISEDKWNKTLQKVSKKLKEHFPNKTIKFEPSSGGDLEITTHSFNCRGEFFYCNTSKLFNSTYNSTNSTITLPCRIKQIINMWQEVGRAMYAPPIAGNITCKSNITGLLLTRDGGKNNTETFRPGGGDMRDNWRSELYKYKVVEIKPLGIAPTKAKRRVVEREKRAVGIGAVFLGFLGAAGSTMGAASITLTVQARQLLSGIVQQQSNLLRAIEAQQHMLQLTVWGIKQLQTRVLAIERYLKDQQLLGIWGCSGKLICTTAVPWNSSWSNKSQEDIWDNMTWMQWDREISNYTDTIYRLLEDSQNQQEKNEKDLLALDSWKNLWNWFDITNWLWYIKIFIMIVGGLIGLRIIFAVLSIVNRVRQGYSPLSFQTLTPNPRGPDRLGRIEEEGGEQDRDRSIRLVSGFLALAWDDLRSLCLFSYHRLRDFILIAARAVELLGRSSLRGLQRGWEALKYLGSLVQYWGLELKKSAISLLDTIAIAVAEGTDRIIELIQRICRAIRNIPRRIRQGFEAALQ

SEQ ID NO: 47 - protein, 835 aa, Human immunodeficiency virus
MRVMGILRNCQQWWIWGILGFWMLMICNVVGNLWVTVYYGVPVWKEAKTTLFCASDAKAYEREVHNVWATHACVPTDPNPQEMVLENVTENFNMWKNDMVDQMHEDIISLWDQSLKPCVKLTPLCVTLNCTNATNATNTMGEMKNCSFNITTELRDKKQKVYALFYRLDIVPLNDNNSYRLINCNTSAITQACPKVSFDPIPIHYCAPAGYAILKCNNKTFNGTGPCNNVSTVQCTHGIKPVVSTQLLLNGSLAEEEIIIRSENLTDNAKTIIVHLNESVEIVCTRPNNNTRKSIRIGPGQTFYATGDIIGDIRQAHCNISEEKWNKTLQRVGEKLKEHFPNKTIKFAPSSGGDLEITTHSFNCRGEFFYCNTSRLFNSTYNSKNSTITLPCRIKQIINMWQGVGRAMYAPPIAGNITCKSNITGLLLTRDGGKNNTETFRPGGGDMRDNWRSELYKYKVVEIKPLGIAPTEAKRRVVEREKRAVGIGAVFLGFLGAAGSTMGAASITLTVQARQLLSGIVQQQSNLLRAIEAQQHMLQLTVWGIKQLQTRVLAIERYLKDQQLLGIWGCSGKLICTTAVPWNSSWSNKSQEEIWDNMTWMQWDREISNYTDTIYRLLEDSQNQQEKNEQDLLALDSWENLWNWFDITNWLWYIKIFIMIVGGLIGLRIIFAVLSIVNRVRQGYSPLSFQTLTPNPRGPDRLGRIEEEGGEQDRDRSIRLVSGFLALAWDDLRSLCLFSYHRLRDFILIAARAVELLGRSSLRGLQRGWEALKYLGSLVQYWGLELKKSAISLLDTIAIAVAEGTDRIIELIQRICRAIRNIPRRIRQGFEAALL

SEQ ID NO: 48 - protein, 840 aa, Human immunodeficiency virus
MRVRGIQRNYQHLWRWGIMLLGMLMICSVAENLWVTVYYGVPVWKEATTTLFCASDAKSYKTEAHNIWATHACVPTDPNPQEIELENVTENFNMWKNNMVEQMHEDIISLWDQSLKPCVKLTPLCVTLNCTDVKRNNTSNDTNEGEMKNCSFNITTEIRDKKKQVHALFYKLDVVPIDDNNSNTSYRLINCNTSAITQACPKVTFEPIPIHYCAPAGFAILKCKDKKFNGTGPCKNVSTVQCTHGIRPVVSTQLLLNGSLAEEEIIIRSENLTNNAKIIIVQLNESVTINCTRPYNNTRQRTPIGPGQALYTTRIKGDIRQAHCNISRAEWNKTLQQVAKKLGDLLNKTTIIFKPSSGGDPEITTHSFNCGGEFFYCNTSRLFNSTWNNTKWNSTGKITLPCRIKQIINMWQGVGKAMYAPPIEGLIKCSSNITGLLLTRDGGANNSHNETFRPGGGDMRDNWRSELYKYKVVKIEPLGVAPTRAKRRVVEREKRAIGLGAMFLGFLGAAGSTMGAASMTLTVQARQLLSGIVQQQNNLLRAIEAQQHLLQLTVWGIKQLQARILAVERYLKDQQLLGIWGCSGKHICTTTVPWNSSWSNKSLDEIWNNMTWMEWEREIDNYTGLIYSLIEESQNQQEKNEQELLELDKWASLWNWFSITQWLWYIKIFIMIVGGLIGLRIVFAVLSLVNRVRQGYSPLSFQTLLPAPRGPDRPEGIEEEGGEQGRGRSIRLVNGFSALIWDDLRNLCLFSYHRLRDLILIAARIVELLGRRGWEALKYLWNLLQYWIQELKNSAISLFDTTAIAVAEGTDRVIEIVQRACRAILNIPTRIRQGLERALL

SEQ ID NO: 49 - protein, 832 aa, Human immunodeficiency virus
MRVRGMQRNWQHLGKWGLLFLGILIICNAAENLWVTVYYGVPVWKEATTTLFCASDAKSYEKEVHNVWATHACVPTDPNPQEVVLENVTENFDMWKNNMVEQMHTDIISLWDQSLKPCVKLTPLCVTLNCTDVNATNNDTNDNKTGAIQNCSFNMTTEVRDKKLKVHALFYKLDIVPISNNNSKYRLINCNTSTITQACPKVSWDPIPIHYCAPAGYAILKCNDKRFNGTGPCKNVSTVQCTHGIKPVVSTQLLLNGSLAEEDIIIRSQNISDNAKTIIVHLNESVQINCTRPNNNTRKSIHLGPGQAFYATGEIIGDIRKAHCNISGTQWNKTLEQVKAKLKSHFPNKTIKFNSSSGGDLEITMHSFNCRGEFFYCNTSGLFNDTGSNGTITLPCRIKQIVNMWQEVGRAMYAAPIAGNITCNSNITGLLLTRDGGQNNTETFRPGGGNMKDNWRSELYKYKVVEIEPLGVAPTKAKRQVVKRERRAVGIGAVFLGFLGAAGSTMGAASITLTVQARQLLSGIVQQQNNLLRAIEAQQHLLQLTVWGIKQLQARVLAVERYLKDQQLLGLWGCSGKLICTTNVPWNSSWSNKSQDEIWNNMTWMEWEKEISNYSNIIYRLIEESQNQQEKNEQELLALDKWASLWNWFDISNWLWYIKIFIMIVGGLIGLRIVFAVLSIVNRVRKGYSPLSLQTLIPSPREPDRPEGIEEGGGEQGKDRSVRLVNGFLALVWDDLRNLCLFSYRHLRDFILIAARIVDRGLRRGWEALKYLGNLTQYWSQELKNSAISLLNTTAIVVAEGTDRVIEALQRAGRAVLNIPRRIRQGLERALL

SEQ ID NO: 50 - protein, 831 aa, Human immunodeficiency virus
MRVREMQRNWQHLGKWGLLFLGILIICNAADNLWVTVYYGVPVWKEATTTLFCASDAKAYEREVHNVWATYACVPTDPSPQELVLGNVTENFNMWKNNMVDQMHEDIISLWDQSLKPCVKLTPLCVTLNCTDVNVTINTTNVTLGEIKNCSFNITTEIKDKKKKEYALFYRLDVVPINNSIVYRLISCNTSTVTQACPKVSFEPIPIHYCAPAGFAILKCNDKKFNGTGLCRNVSTVQCTHGIRPVVSTQLLLNGSLAEEDIIIRSENISDNTKTIIVQFNRSVEINCTRPNNNTRKSIRIGPGRAFYATGDIIGDIRKAYCNINRTLWNETLKKVAEEFKNHFNITVTFNPSSGGDLEITTHSFNCRGEFFYCNTSDLFNNTEVNNTKTITLPCRIRQFVNMWQRVGRAMYAPPIAGQIQCNSNITGLLLTRDGGKNGSETLRPGGGDMRDNWRSELYKYKVVKIEPLGVAPTKAKRQVVQREKRAVGIGAVLLGFLGAAGSTMGAASITLTVQARQLLSGIVQQQSNLLKAIEAQQHLLQLTVWGIKQLQARILAVERYLKDQQLLGIWGCSGKLICTTNVPWNSSWSNKSQDEIWDNMTWMQWEKEISNYTDTIYRLIEDAQNQQEKNEQDLLALDKWDNLWSWFTITNWLWYIKIFIMIVGGLIGLRIVFAVLSVVNRVRQGYSPLSLQTLIPNPRGPERPGGIEEEGGEQDRDRSIRLVSGFLALAWDDLRSLCLFSYRHLRDFILIAARTVDMGLKRGWEALKYLWNLPQYWGQELKNSAISLLDTTAIAVAEGTDRIIEVLQRAGRAVLHIPRRIRQGFERALL

SEQ ID NO: 51 - protein, 842 aa, Human immunodeficiency virus
MRVKGIQRNWQHLWKWGTLILGLVIICSASNNLWVTVYYGVPVWEDADTTLFCASDAKAYSTERHNVWATHACVPTDPNPQEITLENVTENFNMWKNNMVEQMHEDIISLWDESLKPCVKLTPLCVTLNCTDVNVTNNNTNNTKKEIKNCSFNITTEIRDKKKKEYALFYRLDVVPINDNGNSSIYRLINCNVSTIKQACPKVTFDPIPIHYCAPAGFAILKCRDKKFNGTGPCKNVSTVQCTHGIKPVVSTQLLLNGSLAEEEIIIRSENITDNTKVIIVQLNETIEINCTRPNNNTRKSIRIGPGQAFYATGDIIGDIRQAHCNVSRTKWNEMLQKVKAQLKKIFNKSITFNSSSGGDLEITTHSFNCRGEFFYCNTSGLFNNSLLNSTNSTITLPCKIKQIVRMWQRVGQAMYAPPIAGNITCRSNITGLLLTRDGGNNNTETFRPGGGDMRDNWRSELYKYKIVKIKPLGVAPTRARRRVVEREKRAVGLGAVLLGFLGAAGSTMGAASITLTVQVRQLLSGIVQQQSNLLRAIEAQQHLLQLTVWGIKQLQARVLAVERYLKDQQLLGIWGCSGKLICTTNVPWNTSWSNKSYNEIWDNMTWIEWEREISNYTQQIYSLIEESQNQQEKNEQDLLALDKWASLWNWFDITKWLWYIKIFIMIVGGLIGLRIVFAVLSIVNRVRQGYSPLSFQTLTHHQREPDRPERIEEGGGEQDKDRSIRLVSGFLALAWDDLRSLCLFSYHRLRDFILIAARTVELLGRSSLKGLRLGWEGLKYLWNLLLYWGQELKNSAINLLDTIAIAVANWTDRVIEVAQRACRAILNIPRRIRQGLERALL

SEQ ID NO: 52 - protein, 839 aa, Human immunodeficiency virus
TRVMETQRNYPSLWRWGTLILGMLLICSAAGNLWVTVYYGVPVWKEAKTTLFCASDAKAYETEKHNVWATHACVPTDPNPQEMVLENVTENFNMWENDMVEQMHTDIISLWDQSLKPCVKLTPLCVTLDCSNVNTTNATNSRFNMQEELTNCSFNVTTVIRDKQQKVHALFYRLDVVPIDDNNSYQYRLINCNTSVITQACPKVSFEPIPIHYCAPAGFAILKCNNKTFNGTGPCTNVSTVQCTHGIRPVVSTQLLLNGSLAEEQVIIRSKNISDNTKNIIVQLNKPVEITCTRPNNNTRKSIHLGPGQAFYATGDIIGDIRQAHCNISGKKWNKTLHQVVTQLGKYFDNRTIIFKPHSGGDMEVTTHSFNCRGEFFYCNTSGLFNSSWTNSTNDTKNIITLPCRIKQIVNMWQRVGQAMYAPPIKGNITCVSNITGLILTFDEGNNTVTFRPGGGDMRDNWRSELYKYKVVKIEPLGVAPTEARRRVVEREKRAVGMGAFFLGFLGAAGSTMGAASITLTVQARQLLSGIVQQQSNLLRAIQAQQHMLQLTVWGIKQLQARVLAVERYLKDQQLLGIWGCSGKLICTTNVPWNSSWSNKSLDEIWDNMTWMEWDKQINNYTEEIYRLLEVSQTQQEKNEQDLLALDKWASLWNWFSITNWLWYIKIFIMIVGGLIGLRIIFAVLSIVNRVRQGYSPLSFQTLIPNPRGPDRPEGIEEEGGEQDRDRSVRLVNGFLPLVWDDLRSLCLFSYRLLRDLLLIVVRTVELLGRRGREALKYLWNLLQYWGQELKNSAINLLNTTAIAVAEGTDRIIEIVQRAWRAILHIPRRIRQGFERTLL

SEQ ID NO: 53 - protein, 854 aa, Human immunodeficiency virus
MRVKETQMNWPNLWKWGTLILGLVIICSASDNLWVTVYYGVPVWRDADTTLFCASDAKAHETEVHNVWATHACVPTDPNPQEIHLENVTENFNMWKNNMVEQMQEDVISLWDQSLKPCVKLTPLCVTLNCTNANLTNVNNITNVSNIIGNITNEVRNCSFNMTTELRDKKQKVHALFYKLDIVQIEDNNSYRLINCNTSVIKQACPKISFDPIPIHYCTPAGYAILKCNDKNFNGTGPCKNVSSVQCTHGIKPVVSTQLLLNGSLAEEEIIIRSENLTNNAKTIIVHLNKSVEINCTRPSNNTRTSITIGPGQVFYRTGDIIGDIRKAYCEINGTKWNEVLKQVTEKLKEHFNNKTIIFQPPSGGDLEITMHHFNCRGEFFYCNTTKLFNNTCIGNETMEGCNGTIILPCKIKQIINMWQGAGQAMYAPPISGRINCVSNITGILLTRDGGANNTNETFRPGGGNIKDNWRSELYKYKVVQIEPLGIAPTRAKRRVVEREKRAVGIGAMIFGFLGAAGSTMGAASITLTVQARQLLSGIVQQQSNLLRAIEAQQHLLQLTVWGIKQLQARVLAVERYLKDQKFLGLWGCSGKIICTTAVPWNSTWSNRSFEEIWNNMTWIEWEREISNYTNQIYEILTESQNQQDRNEKDLLELDKWASLWNWFDITNWLWYIKIFIMIVGGLIGLRIIFAVLSIVNRVRQGYSPLSFQTPTHHQREPDRPERIEEGGGEQGRDRSVRLVSGFLALAWDDLRSLCLFSYHRLRDFILIAARTVELLGHSSLKGLRRGWEGLKYLGNLLLYWGQELKISAISLLDATAIAVAGWTDRVIEVAQGAWRAILHIPRRIRQGLERALL

SEQ ID NO: 54 - protein, 844 aa, Human immunodeficiency virus type 1
MRVMGIQKNYPLLWRWGMIIFWIMIICNAENLWVTVYYGVPVWRDAETTLFCASDAKAYDTEVHNVWATHACVPTDPNPQEIHLENVTENFNMWKNNMVEQMHEDIISLWDQSLKPCVKLTPLCVTLDCHNNITNSNTTNNNAGEIKNCSFNMTTELRDKKQKVYALFYRLDVVQINKNNSQYRLINCNTSAITQACPKVSFEPIPIHYCAPAGFAILKCNDKEFNGTGPCKNVSTVQCTHGIKPVVSTQLLLNGSLAEEEIVIRSENITNNAKTIIVQLVKPVKINCTRPNNNTRKSVRIGPGQTFYATGDIIGDIRQAHCNVSRTKWNNTLQQVATQLRKYFNKTIIFANPSGGDLEITTHSFNCGGEFFYCNTSELFNSTWNSTWNNTEKCITLQCRIKQIVNMWQKVGQAMYAPPIQGVIRCESNITGLLLTRDGGNNNSTNETFRPGGGDMRDNWRSELYKYKVVKIEPLGVAPTRAKRRVVEREKRAVGLGAVFLGFLGAAGSTMGAASITLTVQARQLLSGIVQQQSNLLRAIEAQQHLLKLTVWGIKQLQARVLALERYLKDQQLLGIWGCSGKLICTTTVPWNSSWSNKTYNDIWDNMTWLQWDKEISNYTDIIYNLIEESQNQQEKNEQDLLALDKWASLWNWFDITNWLWYIKIFIMIVGGLIGLRIVFAVLTIINRVRQGYSPLSFQTLTHHQREPDRPERIEEGGGEQDRDRSVRLVSGFLALAWDDLRSLCLFSYHRLRDFVLIAARTVELLGHSSLKGLRLGWEALKYLGNLLSYWGQELKNSAINLLDTIAIAVANWTDRVIEIGQRAGRAILNIPRRIRQGLERALL

SEQ ID NO: 55 - protein, 840 aa, Human immunodeficiency virus
MRVKEIRKHLWRWGTLFLGMLMICSATENLWVTVYYGVPVWKEATTTLFCASDAKAYSKEVHNVWATYACVPTDPSPQEIPLENVTENFNMGKNNMVEQMHEDIISLWDQSLKPCVKLTPLCVTLNCTDLKKNVTSTNTSSIKMMEMKNCSFNITTDLRDKVKKEYALFYKLDVVQIDNDSYRLISCNTSVVTQACPKISFEPIPIHYCAPAGFAILKCNDKKFNGTGPCTNVSTVQCTHGIKPVVSTQLLLNGSLAEEEVVIRSVNFTDNTKTIIVQLKEPVEINCTRPNNNTRKGIHIGPGRAFYATGDIIGDIRQAHCNISITKWNNTLKQIVIKLRKQFGNKTIVFNQSSGGDPEIVMHSFNCGGEFFYCNTTKLFNSTWNGTEELNNTEGDIVTLPCRIKQIINMWQEVGKAMYAPPIAGQIRCSSNITGLLLTRDGGNQSNVTEIFRPGGGDMRDNWRSELYKYKVVKIEPLGVAPTKAKRRVVQREKRAVGIGAVFLGFLGAAGSTMGAASITLTVQARQLLSGIVQQQNNLLRAIEAQQHLLQLTVWGIKQLQARVLAVERYLKDQQLLGIWGCSGKLICTTAVPWNTSWSNKSLDEIWNNMTWMEWEREINNYTGLIYNLIEESQNQQEKNEQEILALDKWASLWNWFDISKWLWYIKIFIMIVGGLVGLRIIFAVLSIVNRVRQGYSPLSFQTRLPTQRGPDRPEGIEEEGGERDRDTSIRLVNGFLALIWDDLRSLCLFIYHHLRDLLLIAARIVELLGRRGWEALKYWWNLLQYWIQELKSSAINLIDTIAIAVAGWTDRVIEIGQRFCRAIRNIPRRIRQGAEKALQ

SEQ ID NO: 56 - protein, 848 aa, Human immunodeficiency virus
MRVMGIQRNYPHLWEWGTLILGLVIICSASKNLWVTVYYGVPVWRDAETTPFCASDAKAYDKEVHNIWATHACVPTDPNPQEIALKNVTENFNMWKNNMVEQMHEDIISLWDEGLKPCVKLTPLCVALNCSNATINNSTKTNSTEEIKNCSFNITTEIRDKKKKEYALFYRLDIVPINDSANNNSINSEYMLINCNASTIKQACPKVTFEPIPIHYCAPAGFAILKCNDKNFTGLGPCTNVSSVQCTHGIKPVVSTQLLLNGSLATEGVVIRSKNFTDNTKNIIVQLAKAVKINCTRPNNNTRKSVHIGPGQTWYATGEIIGDIRQAHCNISGNDWNETLQKIVEELRKHFPNKTIIFAPSAGGDLEITTHSFNCGGEFFYCNTSELFNSTYMNSTNSTTINKTITLPCRIKQIVSMWQEVGQAMYAPPIAGSINCSSDITGIILTRDGGNNNTNNETFRPGGGDMRDNWRSELYKYKVVKIEPVGVAPTRARRRVVQREKRAVGIGAVFLGFLGAAGSTMGAASITLTVQARQLLSGIVQQQSNLLRAIEAQQHLLRLTVWGIKQLQARVLALESYLKDQQLLGIWGCSGKLICTTNVPWNSSWSNKSYNDIWDNMTWLQWDKEINNYTQIIYELLEESQNQQEKNEQDLLALDKWANLWNWFNISNWLWYIKIFIMIVGGLIGLRIIFAVLSIVNRVRQGYSPLSLQTLIPTTQRGPDRPEGTEEEGGEQDRSRSIRLVNGFLPLIWDDLRNLCLFSYRHLRNLLLIVARTVELLGIRGWEALKYLWNLLLYWGQELRNSAINLLDTTAIAVAEGTDRIIEAVQRACRAIRNIPRRIRQGLERALL

SEQ ID NO: 57 - protein, 832 aa, Human immunodeficiency virus
MRVKGIQKNWQHLWKWGTLILGLVIICSASNNMWVTVYYGVPAWEDADTILFCASDAKAYSAEKHNVWATHACVPTDPNPQEIALENVTENFNMWKNHMVEQMHEDIISLWDESLKPCVKLTPLCVTLNCTNVTKNNNTKIMGREEIKNCSFNVTTEIRDKKKKEYALFYRLDVVPIDDNNNSYRLINCNASTIKQACPKVSFEPIPIHYCAPAGFAILKCRDKNFNGTGPCKNVSTVQCTHGIKPVVSTQLLLNGSLAEEEIIIKSENLTDNTKTIIVQLNKSVEIRCTRPNNNTRKSISFGPGQAFYATGDIIGDIRQAHCNVSRTDWNNMLQNVTAKLKELFNKNITFNSSAGGDLEITTHSFNCGGEFFYCNTSQLFNSTRPNETNTITLPCKIKQIVRMWQRVGQAMYAPPIAGNITCTSNITGLLLTRDGNNNDSETFRPGGGDMRDNWRSELYKYKVVKIKPLGIAPTRARRRVVGREKRAVGLGAVFLGFLGTAGSTMGAASITLTVQVRQLLSGIVQQQSNLLRAIEAQQHLLQLTVWGIKQLQARVLAVERYLKDQQLLGIWGCSGKLICPTNVPWNASWSNKTYNEIWDNMTWIEWDREINNYTQQIYSLIEESQNQQEKNEQDLLALDKWASLWSWFDISNWLWYIKIFIMIVGGLIGLRIVFAVLSIVNRVRQGYSPLSLQTLIPNPTGADRPGEIEEGGGEQGRTRSIRLVNGFLALAWDDLRSLCLFSYHRLRDFVLIAARTVETLGHRGWEILKYLGNLVCYWGQELKNSAISLLDTTAIAVANWTDRVIEVVQRVFRAFLNIPRRIRQGFERALL

SEQ ID NO: 58 - protein, 858 aa, Human immunodeficiency virus
MRVRGTRRNYQQWWIWGVLGFWMLMICNVEGNLWVTVYYGVPVWKEAKTTLFCASDAKAYETEVHNVWATHACVPTDPNPQEIVMENVTENFNMWNNDMVNQMHEDVISLWDQSLKPCVKLTPLCVTLECTNVSSNGNGTYNETYNESVKEIKNCSFNATTLLRDRKKTVYALFYRLDIVPLNDENSGKNSSEYYRLINCNTSAITQACPKVTFDPIPIHYCTPAGYAILKCNDKKFNGTGQCHNVSTVQCTHGIKPVVSTQLLLNGSLAEREIIIRSENLTNNVKTIIVHLNQSVEIVCTRPNNNTRKSIRIGPGQTFYATGDIIGDIRQAHCNISKDKWYETLQRVSKKLAEHFPNKTIKFASSSGGDLEITTHSFNCRGEFFYCNTSGLFNGTYMNGTNNSSSIITIPCRIKQIINMWQEVGRAMYAPPIEGNITCKSNITGLLLVRDGGRTESNNTEIFRPGGGDMRNNWRNELYKYKVVEIKPLGVAPTAAKRRVVEREKRAVGLGAVFLGFLGAAGSTMGAASITLTVQARQLLSGIVQQQSNLLRAIEAQQHMLQLTVWGIKQLQTRVLAIERYLKDQQLLGIWGCSGKLICTTAVPWNSSWSNKSQQEIWDNMTWMQWDKEISNYTNTIYRLLEDSQNQQERNEKDLLALDSWKNLWSWFDITNWLWYIKIFIMIVGGLIGLRIIFAVLSIVNRVRQGYSPLSFQILTPNPGGPGRLGRIEEEGGEQDKTRSIRLVNGFLALAWDDLRNLCLFSYHRLRDFILLTARGVELLGRNSLRGLQRGWEALKYLGSLVQYWGLELKKSTISLVDTIAIAVAEGTDRIINIVQGICRAIHNIPRRIRQGFEAALQ

SEQ ID NO: 59 - protein, 837 aa, Human immunodeficiency virus
MRVMGIQRNCQQWWIWGILGFWMLMICNATGNLWVTVYYGVPVWKETTTTLFCASDAKAYKAEAHNIWATHACVPTDPNPQEIVLENVTENFNMWKNGMVDQMHEDIISLWDQGLKPCVKLTPLCVTLNCSDVNATNSATNTVVAGMKNCSFNITTEIRDKKKQEYALFYKLDVVQIDGSNTSYRLINCNTSAITQACPKVTFEPIPIHYCAPAGFAILKCNDKKFNGTGPCKNVSTVQCTHGIKPVVSTQLLLNGSLAEEEIIIRSENLTDNAKTIIVQLNESVTINCTRPNNNTRKSIRIGPGQTFYATGDIIGNIRQAYCNISGTEWNKTLQQVAKKLGDLLNKTTIIFKPSSGGDPEITTHTFNCGGEFFYCNTSKLFNSSWTSNNTGNTSTITLPCRIKQIINMWQGVGKAIYAPPIAGLINCSSNITGLLLTRDGGANNSETFRPGGGDMRDNWRSELYKYKVVKIEPLGLAPTKAKRRVVEREKRAIGLGAVFLGFLGAAGSTMGAASLTLTVQARQLLSGIVQQQNNLLRAIEAQQHLLQLTVWGIKQLQARVLAVESYLKDQQLLGIWGCSGKHICTTNVPWNSSWSNKSLEEIWDNMTWMEWEREIDNYTGLIYSLIEESQNQQEKNEQELLQLDKWASLWNWFSITNWLWYIKIFIMIVGGLIGLRIVFAVLSLVNRVRQGYSPLSFQTLLPAPRGPDRPEGIEEEGGEQGRGRSIRLVNGFSALIWDDLRNLCLFSYHRLRDLILIATRIVELLGRRGWEAIKYLWNLLQYWIQELKNSAISLLDTTAIAVAEGTDRAIEIVQRAVRAVLNIPTRIRQGLERALL

SEQ ID NO: 60 - protein, 839 aa, Human immunodeficiency virus
MRVKETQRNWHNLWRWGLMIFGMLMICNATENLWVTVYYGVPVWKDADTTLFCASDAKAYSTEKHNVWATHACVPTDPNPQEIPLENVTENFNMWKNNMVEQMHEDIISLWDESLKPCVKLTPLCVTLNCTDVKNATNTTVEAAEIKNCSFNITTEIKDKKKKEYALFYKLDVVPINDNNNSIYRLINCNVSTVKQACPKVTFEPIPIHYCAPAGFAILKCNDKKFNGTGPCKNVSTVQCTHGIKPVVSTQLLLNGSLAEGEVRIRSENFTNNAKTIIVQLNSSVRINCTRPNNNTRKSIHIGPGQAFYATGDIIGDIRQAHCNISRAEWNNTLQQVAKQLRENFNKTIIFNNPSGGDLEITTHSFNCGGEFFYCNTSRLFNSTWNNDTRNDTKQMHITLPCRIKQIVNMWQRVGQAMYAPPIQGKIRCNSNITGLLLTRDGGNNNTNETFRPTGGDMRDNWRSELYKYKVVEIKPLGVAPTRAKRRVVEREKRAVGIGAVLLGFLGAAGSTMGAASITLTVQARQLLSGIVQQQSNLLKAIEAQQHLLKLTVWGIKQLQARVLAVERYLKDQQLLGIWGCSGKLICTTNVPWNFSWSNKSYDEIWDNMTWIEWEREINNYTQTIYTLLEESQNQQEKNEQDLLALDKWASLWNWFDISNWLWYIKIFIMIVGGLIGLRIIFAVLSIVNRCRQGYSPLSFQTLTPNHKEADRPGGIEEGGGEQDRTRSIRLVSGFLALAWDDLRNLCLFSYHRLRDFILIAARIVETLGRRGWEILKYLGNLAQYWGQELKNSAISLLNATAIAVAEGTDRIIEVVHRVLRAILHIPRRIRQGFERALL

SEQ ID NO: 61 - protein, 838 aa, Human immunodeficiency virus
MRVRGMQRNWQHLGKWGLLFLGILIICNATENLWVTVYYGVPVWKEATTTLFCASDAKSYEREVHNVWATHACVPTDPNPQEVDLENVTENFDMWKNNMVEQMHTDIISLWDQSLKPCVKLTPLCVTLNCTDANATANATKEHPEGRAGAIQNCSFNMTTEVRDKQMKVQALFYRLDIVPISDNNSNEYRLINCNTSTITQACPKVSWDPIPIHYCAPAGYAILKCNDKKFNGTGPCKNVSTVQCTHGIKPVVSTQLLLNGSLAEEEIIIRSQNISDNAKTIIVHLNESVQINCTRPNNNTRKSIHIGPGRAFYATGDIIGDIRKAHCNVSGTQWNKTLEQVKKKLRSYFNTTIKFNSSSGGDPEITMHSFNCRGEFFYCNTSKLFNDTVSNDTIILPCRIKQIVNMWQEVGRAMYAAPIAGNITCTSNITGLLLTRDGGHNETNKTETFRPGGGNMKDNWRSELYKYKVVEIEPLGVAPTRAKRQVVKREKRAVGIGALFLGFLGAAGSTMGAASITLTVQARQLLSGIVQQQSNLLRAIEAQQHLLQLTVWGIKQLQARVLAVERYLKDQQLLGLWGCSGKLICTTNVPWNSSWSNKSQEEIWENMTWMEWEKEINNYSNEIYRLIEESQNQQEKNEQELLALDKWASLWNWFDISNWLWYIRIFIMIVGGLIGLRIVFAVLSIVNRVRKGYSPLSLQTHIPSPREPDRPEGIEEGGGEQGKDRSVRLVNGFLALIWDDLRSLCLFSYHRLRDLLLIVTRIVELLGRRGWEVLKYWWNLLQYWSQELKNSAISLLNTTAIVVAEGTDRVIEALQRVGRAILNIPRRIRQGLERALL

SEQ ID NO: 62 - protein, 855 aa, Human immunodeficiency virus
MKAKGTQRNWQSLWKWGTLILGLVIICSASNDLWVTVYYGVPVWKEATTTLFCASDAKAYDAEVHNVWATHACVPTDPNPQEVALENVTENFNMWENNMVDQMQEDIISLWDQSLKPCVELTPLCVTLNCTDFNNTTNNTTNTRNDGEGEIKNCSFNITTSLRDKIKKEYALFYNLDVVQMDNDNSSYRLTSCNTSIITQACPKVSFTPIPIHYCAPAGFVILKCNNKTFNGTGPCTNVSTVQCTHGIRPVVSTQLLLNGSLAEEEIVIRSKNFTDNAKTIIVQLKDPIEINCTRPNNNTRKRITMGPGRVLYTTGQIIGDIRKAHCNISKTKWNNTLGQIVKKLREQFMNKTIVFQRSSGGDPEIVMHSFNCGGEFFYCNTTQLFNSTWRSNSTWNDTTETNNTDLITLPCRIKQIVNMWQKVGKAMYAPPISGQIRCSSNITGLLLIRDGGSNNTETFRPGGGNMKDNWRSELYKYKVVKIEPLGVAPTRAKRRVVQREKRAVGIGALLFGFLGAAGSTMGAASMTLTVQARQLLSGIVQQQNNLLRAIEAQQHMLQLTVWGIKQLQARVLAVERYLKDQQLLGIWGCSGKLICTTTVPWNASWSNKSLDDIWNNMTWMEWEREIDNYTGLIYTLIEQSQNQQERNEQELLELDKWASLWNWFNITNWLWYIKIFIMIIGGLIGLRIVFAVLSIINRVRKGYSPLSFQTLTHHQREPDRPGRIEEEGGEQDKDRSIRLVSGFLALAWDDLRSLCLFSYHRLRDFILIAARTVELLGRSSLKGLRLGWEGLKYLWNLLLYWGRELKNSAINLLDTVAIAVANWTDRAIEVVQRVGRAVLNIPVRIRQGLERALL

SEQ ID NO: 63 - protein, 22 aa, Human immunodeficiency virus
IFIMIVGGLIGLRIVFAVLSIV

SEQ ID NO: 64 - protein, 22 aa, Human immunodeficiency virus
IFIMIVGGLIGLRIVFAVLSVI

SEQ ID NO: 65 - protein, 22 aa, Human immunodeficiency virus
IFIMIVGGLIGLRIVIAIISVV

SEQ ID NO: 66 - protein, 22 aa, Human immunodeficiency virus
IFIMIVGGLVGLRIVFAVLSIV

SEQ ID NO: 67 - protein, 22 aa, Human immunodeficiency virus
IFIMIVGGLIGLRIIFAVLSIV

SEQ ID NO: 68 - protein, 22 aa, Human immunodeficiency virus
IFIMIVGGLIGLRIVFAVLSLV

SEQ ID NO: 69 - protein, 22 aa, Human immunodeficiency virus
IFIMIVGGLIGLRIVFAVLSVV

SEQ ID NO: 70 - protein, 22 aa, Human immunodeficiency virus
IFIMIVGGLIGLRIVFAVLTII

SEQ ID NO: 71 - protein, 22 aa, Human immunodeficiency virus type 2
IFIMIVGGLVGLRIIFAVLSIV

SEQ ID NO: 72 - protein, 22 aa, Human immunodeficiency virus
IFIMIIGGLIGLRIVFAVLSII

SEQ ID NO: 73 - protein, 12 aa, Synthetic
AEAAAKEAAAKA

SEQ ID NO: 74 - protein, 20 aa, Synthetic
TWIQNPGTKWYQNPGTKIYT

SEQ ID NO: 75 - protein, 8 aa, Synthetic
SGSGASGS

SEQ ID NO: 76 - protein, 4 aa, Synthetic
PSGP

SEQ ID NO: 77 - protein, 216 aa, Synthetic
APNLLGGPSVFIFPPKIKDVLMISLSPIVTCVVVDVSEDDPDVQISWFVNNVEVHTAQTQTHREDYNSTLRVVSALPIQHQDWMSGKEFKCKVNNKDLPAPIERTISKPKGSVRAPQVYVLPPPEEEMTKKQVTLTCMVTDFMPEDIYVEWTNNGKTELNYKNTEPVLDSDGSYFMYSKLRVEKKNWVERNSYSCSVVHEGLHNHHTTKSFSRTPG

SEQ ID NO: 78 - protein, 231 aa, Synthetic
PRGPTIKPCPPCKCPAPNLLGGPSVFIFPPKIKDVLMISLSPIVTCVVVDVSEDDPDVQISWFVNNVEVHTAQTQTHREDYNSTLRVVSALPIQHQDWMSGKEFKCKVNNKDLPAPIERTISKPKGSVRAPQVYVLPPPEEEMTKKQVTLTCMVTDFMPEDIYVEWTNNGKTELNYKNTEPVLDSDGSYFMYSKLRVEKKNWVERNSYSCSVVHEGLHNHHTTKSFSRTPG

SEQ ID NO: 79 - protein, 15 aa, Synthetic
PRGPTIKPCPPCKCP

SEQ ID NO: 80 - protein, 213 aa, Synthetic
VPEVSSVFIFPPKPKDVLTITLTPKVTCVVVDISKDDPEVQFSWFVDDVEVHTAQTQPREEQFNSTFRSVSELPIMHQDWLNGKEFKCRVNSAAFPAPIEKTISKTKGRPKAPQVYTIPPPKEQMAKDKVSLTCMITDFFPEDITVEWQWNGQPAENYKNTQPIMDTDGSYFVYSKLNVQKSNWEAGNTFTCSVLHEGLHNHHTEKSLSHSPG

SEQ ID NO: 81 - protein, 40 aa, Synthetic
KPLDGEYFTLQIRGRERFEMFRELNEALELKDAQAGKEPG

SEQ ID NO: 82 - protein, 27 aa, Synthetic
GYIPEAPRDGQAYVRKDGEWVLLSTFL

SEQ ID NO: 83 - protein, 94 aa, Synthetic
GSHMWKQSVELAKKDSLYKDAMQYASESKDTELAEELLQWFLQEEKRECFGACLFTCYDLLRPDVVLELAWRHNIMDFAMPYFIQVMKEYLTKV

SEQ ID NO: 84 - protein, 20 aa, Synthetic
MYRMQLLSCIALSLALVTNS

SEQ ID NO: 85 - protein, 6 aa, Synthetic
HHHHHH

SEQ ID NO: 86 - protein, 905 aa, Synthetic
MYRMQLLSCIALSLALVTNSGVPVWKDAETTLFCASDAKAYDTEVHNVWATHACVPTDPNPQEIHLENVTEDFNMWKNNMVEQMHTDIISLWDQSLKPCVKLTPLCVTLDCNATASNVTNEMRNCSFNITTELKDKKQQVYSLFYKLDVVQINEKNETDKYRLINCNTSAITQACPKVSFEPIPIHYCAPAGFAILKCKDTEFNGTGPCKNVSTVQCTHGIRPVISTQLLLNGSLAEEGIQIRSENITNNAKTIIVQLDKAVKINCTRPNNNTRKGVRIGPGQAFYATGGIIGDIRQAHCNVSRAKWNDTLRGVAKKLREHFKNKTIIFEKSSGGDIEITTHSFNCGGEFFYCNTSGLFNSTWESNSTESNNTTSNDTITLTCRIKQIINMWQKVGQAMYAPPIQGVIRCESNITGLLLTRDGGNNSTNEIFRPGGGNMRDNWRSELYKYKVVKIEPSGPVPEVSSVFIFPPKPKDVLTITLTPKVTCVVVDISKDDPEVQFSWFVDDVEVHTAQTQPREEQFNSTFRSVSELPIMHQDWLNGKEFKCRVNSAAFPAPIEKTISKTKGRPKAPQVYTIPPPKEQMAKDKVSLTCMITDFFPEDITVEWQWNGQPAENYKNTQPIMDTDGSYFVYSKLNVQKSNWEAGNTFTCSVLHEGLHNHHTEKSLSHSPGIPIVQNLQGQMVHQAISPRTLNAWVKVVEEKAFSPEVIPMFSALSEGATPQDLNTMLNTVGGHQAAMQMLKETINEEAAEWDRVHPVHAGPIAPGQMREPRGSDIAGTTSTLQEQIGWMTNNPPIPVGEIYKRWIILGLNKIVRMYSPTSILDIRQGPKEPFRDYVDRFYKTLRAEQASQDVKNWMTETLLVQNANPDCKTILKALGPAATLEEMMTACQGVGGPGHKARVL

SEQ ID NO: 87 - protein, 914 aa, Synthetic
MYRMQLLSCIALSLALVTNSGVPVWKDAETTLFCASDAKAYDTEVHNVWATHACVPTDPNPQEIHLENVTEDFNMWKNNMVEQMHTDIISLWDQSLKPCVKLTPLCVTLDCNATASNVTNEMRNCSFNITTELKDKKQQVYSLFYKLDVVQINEKNETDKYRLINCNTSAITQACPKVSFEPIPIHYCAPAGFAILKCKDTEFNGTGPCKNVSTVQCTHGIRPVISTQLLLNGSLAEEGIQIRSENITNNAKTIIVQLDKAVKINCTRPNNNTRKGVRIGPGQAFYATGGIIGDIRQAHCNVSRAKWNDTLRGVAKKLREHFKNKTIIFEKSSGGDIEITTHSFNCGGEFFYCNTSGLFNSTWESNSTESNNTTSNDTITLTCRIKQIINMWQKVGQAMYAPPIQGVIRCESNITGLLLTRDGGNNSTNEIFRPGGGNMRDNWRSELYKYKVVKIEVPRDCGCKPCICTVPEVSSVFIFPPKPKDVLTITLTPKVTCVVVDISKDDPEVQFSWFVDDVEVHTAQTQPREEQFNSTFRSVSELPIMHQDWLNGKEFKCRVNSAAFPAPIEKTISKTKGRPKAPQVYTIPPPKEQMAKDKVSLTCMITDFFPEDITVEWQWNGQPAENYKNTQPIMDTDGSYFVYSKLNVQKSNWEAGNTFTCSVLHEGLHNHHTEKSLSHSPGIPIVQNLQGQMVHQAISPRTLNAWVKVVEEKAFSPEVIPMFSALSEGATPQDLNTMLNTVGGHQAAMQMLKETINEEAAEWDRVHPVHAGPIAPGQMREPRGSDIAGTTSTLQEQIGWMTNNPPIPVGEIYKRWIILGLNKIVRMYSPTSILDIRQGPKEPFRDYVDRFYKTLRAEQASQDVKNWMTETLLVQNANPDCKTILKALGPAATLEEMMTACQGVGGPGHKARVL

SEQ ID NO: 88 - protein, 894 aa, Synthetic
MYRMQLLSCIALSLALVTNSGVPVWRNASIPLFCATKNRDTWGTIQCLPDNDDYQEIALNVTEAFDAWNNTVTEQAVEDVWSLFETSIKPCVKLTPLCVAMSCNSTTIPPSEEMVDCQFNMTGLDRDKKKQYNETWYSKDVVCELNKTDGGRGRCYMNHCNTSVITESCDKHYWDAIRFRYCAPPGFALLRCNDTNYSGFMPNCSKVVVSSCTRMMETQTSTWLGFNGTRAENRTYMYWHSKDNRTIISLNKYYNLTMHCKRPGNKTVAPITLMSGLVFHSQPINRRPRQAWCWFKGQWREAMQEVKRTLIKHPRYKGTNDTRNITFTKPGEGSDPEVAYMWTNCRGEFLYCNMTWFLNWVENRTGQTQRNYAPCHIKQIINTWHKVGKNVYLPPREGELTCNSTVTSIIANIDVDSNNNRTNITFSAEVAELYRLELGDYKLIEVTPSGPVPEVSSVFIFPPKPKDVLTITLTPKVTCVVVDISKDDPEVQFSWFVDDVEVHTAQTQPREEQFNSTFRSVSELPIMHQDWLNGKEFKCRVNSAAFPAPIEKTISKTKGRPKAPQVYTIPPPKEQMAKDKVSLTCMITDFFPEDITVEWQWNGQPAENYKNTQPIMDTDGSYFVYSKLNVQKSNWEAGNTFTCSVLHEGLHNHHTEKSLSHSPGIVQQIAGNYVHMPLSPRTLNAWVKLVEEKKFGAEVVPGFQALSEGCTPYDINQMLNCVGDHQAAMQIIREIINEEAADWDQQHPIPGPLPAGQLRDPRGSDIAGTTSTVEEQIQWMYRAQNPVPVGNIYRRWIQIGLQKCVRMYNPTNILDIKQGPKEPFQSYVDRFYKSLRAEQTDPAVKNWMTQTLLIQNANPDCKLVLKGLGMNPTLEEMLTACQGIGGPGQKARLM

SEQ ID NO: 89 - protein, 903 aa, Synthetic
MYRMQLLSCIALSLALVTNSGVPVWRNASIPLFCATKNRDTWGTIQCLPDNDDYQEIALNVTEAFDAWNNTVTEQAVEDVWSLFETSIKPCVKLTPLCVAMSCNSTTIPPSEEMVDCQFNMTGLDRDKKKQYNETWYSKDVVCELNKTDGGRGRCYMNHCNTSVITESCDKHYWDAIRFRYCAPPGFALLRCNDTNYSGFMPNCSKVVVSSCTRMMETQTSTWLGFNGTRAENRTYMYWHSKDNRTIISLNKYYNLTMHCKRPGNKTVAPITLMSGLVFHSQPINRRPRQAWCWFKGQWREAMQEVKRTLIKHPRYKGTNDTRNITFTKPGEGSDPEVAYMWTNCRGEFLYCNMTWFLNWVENRTGQTQRNYAPCHIKQIINTWHKVGKNVYLPPREGELTCNSTVTSIIANIDVDSNNNRTNITFSAEVAELYRLELGDYKLIEVTVPRDCGCKPCICTVPEVSSVFIFPPKPKDVLTITLTPKVTCVVVDISKDDPEVQFSWFVDDVEVHTAQTQPREEQFNSTFRSVSELPIMHQDWLNGKEFKCRVNSAAFPAPIEKTISKTKGRPKAPQVYTIPPPKEQMAKDKVSLTCMITDFFPEDITVEWQWNGQPAENYKNTQPIMDTDGSYFVYSKLNVQKSNWEAGNTFTCSVLHEGLHNHHTEKSLSHSPGIVQQIAGNYVHMPLSPRTLNAWVKLVEEKKFGAEVVPGFQALSEGCTPYDINQMLNCVGDHQAAMQIIREIINEEAADWDQQHPIPGPLPAGQLRDPRGSDIAGTTSTVEEQIQWMYRAQNPVPVGNIYRRWIQIGLQKCVRMYNPTNILDIKQGPKEPFQSYVDRFYKSLRAEQTDPAVKNWMTQTLLIQNANPDCKLVLKGLGMNPTLEEMLTACQGIGGPGQKARLM

SEQ ID NO: 90 - protein, 10 aa, Synthetic
RDCGCKPCIC

SEQ ID NO: 91 - protein, 584 aa, Synthetic
MYRMQLLSCIALSLALVTNSMVFRPGGGDMRDNWRSELYKYKVIKIEPLGIAPTKAKRRVVQREKRQARQLLSGIVQQQNNLLRAIEAQQHLLQLTVWGIKQLQARVLAVERYLRDQQLLGIWGCSGKLICTTAVPWNASWSNKSLEDIWDNMTWMQWEREIDNYTNTIYTLLEESQNQQEKNEQELLGGGGSGGGGSGGGGSVPEVSSVFIFPPKPKDVLTITLTPKVTCVVVDISKDDPEVQFSWFVDDVEVHTAQTQPREEQFNSTFRSVSELPIMHQDWLNGKEFKCRVNSAAFPAPIEKTISKTKGRPKAPQVYTIPPPKEQMAKDKVSLTCMITDFFPEDITVEWQWNGQPAENYKNTQPIMDTDGSYFVYSKLNVQKSNWEAGNTFTCSVLHEGLHNHHTEKSLSHSPGKGGGGSGGGGSGGGGSASMTLTVQARQLLSGIVQQQNNLLRAIEAQQHLLQLTVWGIKQLQARILAVERYLKDQQLLGIWGCSGKLICTTAVPWNASWSNKSLEQIWNHTTWMEWDREINNYTSLIHSLIEESQNQQEKNEQELLELDKWASLWNWFNITNWLWYIKL

SEQ ID NO: 92 - protein, 507 aa, Synthetic
MYRMQLLSCIALSLALVTNSMVFRPGGGDMRDNWRSELYKYKVIKIEPLGIAPTKAKRRVVQREKRQARQLLSGIVQQQNNLLRAIEAQQHLLQLTVWGIKQLQARVLAVERYLRDQQLLGIWGCSGKLICTTAVPWNASWSNKSLEDIWDNMTWMQWEREIDNYTNTIYTLLEESQNQQEKNEQELLGGGGSGGGGSGGGGSGGGGSGGGGSVPEVSSVFIFPPKPKDVLTITLTPKVTCVVVDISKDDPEVQFSWFVDDVEVHTAQTQPREEQFNSTFRSVSELPIMHQDWLNGKEFKCRVNSAAFPAPIEKTISKTKGRPKAPQVYTIPPPKEQMAKDKVSLTCMITDFFPEDITVEWQWNGQPAENYKNTQPIMDTDGSYFVYSKLNVQKSNWEAGNTFTCSVLHEGLHNHHTEKSLSHSPGKGGGGSGGGGSGGGGSGGGGSGGGGSASMTLTVQARQLLSGIVQQQNNLLRAIEAQQHLLQLTVWGIKQLQARILAVERYL

SEQ ID NO: 93 - protein, 604 aa, Synthetic
MYRMQLLSCIALSLALVTNSMASMTLTVQARQLLSGIVQQQNNLLRAIEAQQHLLQLTVWGIKQLQARILAVERYLKDQQLLGIWGCSGKLICTTAVPWNASWSNKSLEQIWNHTTWMEWDREINNYTSLIHSLIEESQNQQEKNEQELLELDKWASLWNWFNITNWLWYIKLGGGGSGGGGSGGGGSGGGGSGGGGSVPEVSSVFIFPPKPKDVLTITLTPKVTCVVVDISKDDPEVQFSWFVDDVEVHTAQTQPREEQFNSTFRSVSELPIMHQDWLNGKEFKCRVNSAAFPAPIEKTISKTKGRPKAPQVYTIPPPKEQMAKDKVSLTCMITDFFPEDITVEWQWNGQPAENYKNTQPIMDTDGSYFVYSKLNVQKSNWEAGNTFTCSVLHEGLHNHHTEKSLSHSPGKGGGGSGGGGSGGGGSGGGGSGGGGSVFRPGGGDMRDNWRSELYKYKVIKIEPLGIAPTKAKRRVVQREKRQARQLLSGIVQQQNNLLRAIEAQQHLLQLTVWGIKQLQARVLAVERYLRDQQLLGIWGCSGKLICTTAVPWNASWSNKSLEDIWDNMTWMQWEREIDNYTNTIYTLLEESQNQQEKNEQELL

SEQ ID NO: 94 - protein, 604 aa, Synthetic
MYRMQLLSCIALSLALVTNSMIFRPGGGNMRDNWRSELYKYKVVKIEPLGVAPSRAKRRVVEREKRQARQLLSGIVQQQSNLLRAIEAQQHMLKLTVWGIKQLQARVLAVERYLKDQQLLGIWGCSGKLICTTNVPWNSSWSNKSMNEIWDNMTWLQWDKEISNYTQIIYNLIEESQNQQEKNEQDLLGGGGSGGGGSGGGGSGGGGSGGGGSVPEVSSVFIFPPKPKDVLTITLTPKVTCVVVDISKDDPEVQFSWFVDDVEVHTAQTQPREEQFNSTFRSVSELPIMHQDWLNGKEFKCRVNSAAFPAPIEKTISKTKGRPKAPQVYTIPPPKEQMAKDKVSLTCMITDFFPEDITVEWQWNGQPAENYKNTQPIMDTDGSYFVYSKLNVQKSNWEAGNTFTCSVLHEGLHNHHTEKSLSHSPGKGGGGSGGGGSGGGGSGGGGSGGGGSASMTLTVQARQLLSGIVQQQNNLLRAIEAQQHLLQLTVWGIKQLQARILAVERYLKDQQLLGIWGCSGKLICTTAVPWNASWSNKSLEQIWNHTTWMEWDREINNYTSLIHSLIEESQNQQEKNEQELLELDKWASLWNWFNITNWLWYIKL

SEQ ID NO: 95 - protein, 604 aa, Synthetic
MYRMQLLSCIALSLALVTNSMTFRPGGGNIKDNWRSELYKYKVVQIEPLGIAPTKAKRRVVEREKRQARQLLSGIVQQQSNLLRAIEAQQHLLQLTVWGIKQLQARVLAVERYLKDQQFLGLWGCSGKIICTTAVPWNSTWSNRSYEEIWNNMTWIEWEREISNYTNQIYEILTESQDQQDRNEKDLLGGGGSGGGGSGGGGSGGGGSGGGGSVPEVSSVFIFPPKPKDVLTITLTPKVTCVVVDISKDDPEVQFSWFVDDVEVHTAQTQPREEQFNSTFRSVSELPIMHQDWLNGKEFKCRVNSAAFPAPIEKTISKTKGRPKAPQVYTIPPPKEQMAKDKVSLTCMITDFFPEDITVEWQWNGQPAENYKNTQPIMDTDGSYFVYSKLNVQKSNWEAGNTFTCSVLHEGLHNHHTEKSLSHSPGKGGGGSGGGGSGGGGSGGGGSGGGGSASMTLTVQARQLLSGIVQQQNNLLRAIEAQQHLLQLTVWGIKQLQARILAVERYLKDQQLLGIWGCSGKLICTTAVPWNASWSNKSLEQIWNHTTWMEWDREINNYTSLIHSLIEESQNQQEKNEQELLELDKWASLWNWFNITNWLWYIKL

SEQ ID NO: 96 - protein, 604 aa, Synthetic
MYRMQLLSCIALSLALVTNSMTFRPGGGDMRDNWRSELYKYKVVKIEPLGVAPTHAKRRVVEREKRQARQLLSGIVQQQSNLLKAIEAQQHLLKLTVWGIKQLQARVLALERYLKDQQLLGIWGCSGKLICTTTVPWNSSWSNKTYNDIWDNMTWLQWDKEISNYTNIIYNLIEESQNQQEKNEQDLLGGGGSGGGGSGGGGSGGGGSGGGGSVPEVSSVFIFPPKPKDVLTITLTPKVTCVVVDISKDDPEVQFSWFVDDVEVHTAQTQPREEQFNSTFRSVSELPIMHQDWLNGKEFKCRVNSAAFPAPIEKTISKTKGRPKAPQVYTIPPPKEQMAKDKVSLTCMITDFFPEDITVEWQWNGQPAENYKNTQPIMDTDGSYFVYSKLNVQKSNWEAGNTFTCSVLHEGLHNHHTEKSLSHSPGKGGGGSGGGGSGGGGSGGGGSGGGGSASMTLTVQARQLLSGIVQQQNNLLRAIEAQQHLLQLTVWGIKQLQARILAVERYLKDQQLLGIWGCSGKLICTTAVPWNASWSNKSLEQIWNHTTWMEWDREINNYTSLIHSLIEESQNQQEKNEQELLELDKWASLWNWFNITNWLWYIKL

SEQ ID NO: 97 - protein, 507 aa, Synthetic
MYRMQLLSCIALSLALVTNSMIFRPGGGDMRDNWRSELYKYKVVKIEPLGVAPTKAKRRVVEREKRQARQLLSGIVQQQNNLLRAIEAQQHLLQLTVWGIKQLQARVLAVERYLKDQQLLGLWGCSGKLICTTAVPWNSSWSNKSMEDIWDNMTWLEWDREISNYTQIIYNLIEESQNQQEKNEQDLLGGGGSGGGGSGGGGSGGGGSGGGGSVPEVSSVFIFPPKPKDVLTITLTPKVTCVVVDISKDDPEVQFSWFVDDVEVHTAQTQPREEQFNSTFRSVSELPIMHQDWLNGKEFKCRVNSAAFPAPIEKTISKTKGRPKAPQVYTIPPPKEQMAKDKVSLTCMITDFFPEDITVEWQWNGQPAENYKNTQPIMDTDGSYFVYSKLNVQKSNWEAGNTFTCSVLHEGLHNHHTEKSLSHSPGKGGGGSGGGGSGGGGSGGGGSGGGGSASMTLTVQARQLLSGIVQQQNNLLRAIEAQQHLLQLTVWGIKQLQARILAVERYL

SEQ ID NO: 98 - protein, 684 aa, Synthetic
MYRMQLLSCIALSLALVTNSMVFRPGGGDMRDNWRSELYKYKVIKIEPLGIAPTKAKRRVVQREKRQARQLLSGIVQQQNNLLRAIEAQQHLLQLTVWGIKQLQARVLAVERYLRDQQLLGIWGCSGKLICTTAVPWNASWSNKSLEDIWDNMTWMQWEREIDNYTNTIYTLLEESQNQQEKNEQELLGGGGSGGGGSGGGGSGGGGSGGGGSVPEVSSVFIFPPKPKDVLTITLTPKVTCVVVDISKDDPEVQFSWFVDDVEVHTAQTQPREEQFNSTFRSVSELPIMHQDWLNGKEFKCRVNSAAFPAPIEKTISKTKGRPKAPQVYTIPPPKEQMAKDKVSLTCMITDFFPEDITVEWQWNGQPAENYKNTQPIMDTDGSYFVYSKLNVQKSNWEAGNTFTCSVLHEGLHNHHTEKSLSHSPGKGGGGSGGGGSGGGGSGGGGSGGGGSMPIVQNLQGQMVHQAISPRTLNAWVKVVEEKAFSPEVIPMFSALSEGATPQDLNTMLNTVGGHQAAMQMLKETINEEAAEWDRVHPVHAGPIAPGQMREPRGSDIAGTTSTLQEQIGWMTNNPPIPVGEIYKRWIILGLNKIVRMYSPTSILDIRQGPKEPFRDYVDRFYKTLRAEQASQDVKNWMTETLLVQNANPDCKTILKALGPAATLEEMMTACQGVGGPGHKARVL

SEQ ID NO: 99 - protein, 684 aa, Synthetic
MYRMQLLSCIALSLALVTNSMPIVQNLQGQMVHQAISPRTLNAWVKVVEEKAFSPEVIPMFSALSEGATPQDLNTMLNTVGGHQAAMQMLKETINEEAAEWDRVHPVHAGPIAPGQMREPRGSDIAGTTSTLQEQIGWMTNNPPIPVGEIYKRWIILGLNKIVRMYSPTSILDIRQGPKEPFRDYVDRFYKTLRAEQASQDVKNWMTETLLVQNANPDCKTILKALGPAATLEEMMTACQGVGGPGHKARVLGGGGSGGGGSGGGGSGGGGSGGGGSVPEVSSVFIFPPKPKDVLTITLTPKVTCVVVDISKDDPEVQFSWFVDDVEVHTAQTQPREEQFNSTFRSVSELPIMHQDWLNGKEFKCRVNSAAFPAPIEKTISKTKGRPKAPQVYTIPPPKEQMAKDKVSLTCMITDFFPEDITVEWQWNGQPAENYKNTQPIMDTDGSYFVYSKLNVQKSNWEAGNTFTCSVLHEGLHNHHTEKSLSHSPGKGGGGSGGGGSGGGGSGGGGSGGGGSMVFRPGGGDMRDNWRSELYKYKVIKIEPLGIAPTKAKRRVVQREKRQARQLLSGIVQQQNNLLRAIEAQQHLLQLTVWGIKQLQARVLAVERYLRDQQLLGIWGCSGKLICTTAVPWNASWSNKSLEDIWDNMTWMQWEREIDNYTNTIYTLLEESQNQQEKNEQELL

SEQ ID NO: 100 - protein, 642 aa, Synthetic
MYRMQLLSCIALSLALVTNSMVFRPGGGDMRDNWRSELYKYKVIKIEPLGIAPTKAKRRVVQREKRQARQLLSGIVQQQNNLLRAIEAQQHLLQLTVWGIKQLQARVLAVERYLRDQQLLGIWGCSGKLICTTAVPWNASWSNKSLEDIWDNMTWMQWEREIDNYTNTIYTLLEESQNQQEKNEQELLGGGGSGGGGSGGGGSGGGGSGGGGSVPEVSSVFIFPPKPKDVLTITLTPKVTCVVVDISKDDPEVQFSWFVDDVEVHTAQTQPREEQFNSTFRSVSELPIMHQDWLNGKEFKCRVNSAAFPAPIEKTISKTKGRPKAPQVYTIPPPKEQMAKDKVSLTCMITDFFPEDITVEWQWNGQPAENYKNTQPIMDTDGSYFVYSKLNVQKSNWEAGNTFTCSVLHEGLHNHHTEKSLSHSPGKGGGGSGGGGSGGGGSGGGGSGGGGSMPIVQNLQGQMVHQAISPRTLNAWVKVVEEKAFSPEVIPMFSALSGGGGSGGGGSGGGGSGGGGSGGGGSMQMLKETINEEAAEWDRVHPVHAGPGGGGSGGGGSGGGGSGGGGSGGGGSQASQDVKNWMTGGGGSGGGGSGGGGSGGGGSGGGGSCKTILKALGPAATLEEMMTACQGVGGPGHKARVL

SEQ ID NO: 101 - protein, 642 aa, Synthetic
MYRMQLLSCIALSLALVTNSMPIVQNLQGQMVHQAISPRTLNAWVKVVEEKAFSPEVIPMFSALSGGGGSGGGGSGGGGSGGGGSGGGGSMQMLKETINEEAAEWDRVHPVHAGPGGGGSGGGGSGGGGSGGGGSGGGGSQASQDVKNWMTGGGGSGGGGSGGGGSGGGGSGGGGSCKTILKALGPAATLEEMMTACQGVGGPGHKARVLGGGGSGGGGSGGGGSGGGGSGGGGSVPEVSSVFIFPPKPKDVLTITLTPKVTCVVVDISKDDPEVQFSWFVDDVEVHTAQTQPREEQFNSTFRSVSELPIMHQDWLNGKEFKCRVNSAAFPAPIEKTISKTKGRPKAPQVYTIPPPKEQMAKDKVSLTCMITDFFPEDITVEWQWNGQPAENYKNTQPIMDTDGSYFVYSKLNVQKSNWEAGNTFTCSVLHEGLHNHHTEKSLSHSPGKGGGGSGGGGSGGGGSGGGGSGGGGSMVFRPGGGDMRDNWRSELYKYKVIKIEPLGIAPTKAKRRVVQREKRQARQLLSGIVQQQNNLLRAIEAQQHLLQLTVWGIKQLQARVLAVERYLRDQQLLGIWGCSGKLICTTAVPWNASWSNKSLEDIWDNMTWMQWEREIDNYTNTIYTLLEESQNQQEKNEQELL

SEQ ID NO: 102 - protein, 684 aa, Synthetic
MYRMQLLSCIALSLALVTNSMVFRPGGGDMRDNWRSELYKYKVIKIEPLGIAPTKAKRRVVQREKRQARQLLSGIVQQQNNLLRAIEAQQHLLQLTVWGIKQLQARVLAVERYLRDQQLLGIWGCSGKLICTTAVPWNASWSNKSLEDIWDNMTWMQWEREIDNYTNTIYTLLEESQNQQEKNEQELLGGGGSGGGGSGGGGSGGGGSGGGGSVPEVSSVFIFPPKPKDVLTITLTPKVTCVVVDISKDDPEVQFSWFVDDVEVHTAQTQPREEQFNSTFRSVSELPIMHQDWLNGKEFKCRVNSAAFPAPIEKTISKTKGRPKAPQVYTIPPPKEQMAKDKVSLTCMITDFFPEDITVEWQWNGQPAENYKNTQPIMDTDGSYFVYSKLNVQKSNWEAGNTFTCSVLHEGLHNHHTEKSLSHSPGKGGGGSGGGGSGGGGSGGGGSGGGGSMPIVQNLQGQMVHQAISPRTLNAWVKVVEEKAFSPEVIPMFSALSQGATPQEVNTVLNTQGGHQAAMQMLKETINEEAAEWDRVHPVHAGPVAPGQVKDPKGSEVAGTTSTVQDQMGWITNNPPVPIGNVQRKWIVVGVNRVVKVYSPTSVLDVKQGPRDPFREYIEKFYRTLKASQASQDVKNWMTDTVVIQNANPECKTILKALGPAATLEEMMTACQGVGGPGHKARVL

SEQ ID NO: 103 - protein, 684 aa, Synthetic
MYRMQLLSCIALSLALVTNSMPIVQNLQGQMVHQAISPRTLNAWVKVVEEKAFSPEVIPMFSALSQGATPQEVNTVLNTQGGHQAAMQMLKETINEEAAEWDRVHPVHAGPVAPGQVKDPKGSEVAGTTSTVQDQMGWITNNPPVPIGNVQRKWIVVGVNRVVKVYSPTSVLDVKQGPRDPFREYIEKFYRTLKASQASQDVKNWMTDTVVIQNANPECKTILKALGPAATLEEMMTACQGVGGPGHKARVLGGGGSGGGGSGGGGSGGGGSGGGGSVPEVSSVFIFPPKPKDVLTITLTPKVTCVVVDISKDDPEVQFSWFVDDVEVHTAQTQPREEQFNSTFRSVSELPIMHQDWLNGKEFKCRVNSAAFPAPIEKTISKTKGRPKAPQVYTIPPPKEQMAKDKVSLTCMITDFFPEDITVEWQWNGQPAENYKNTQPIMDTDGSYFVYSKLNVQKSNWEAGNTFTCSVLHEGLHNHHTEKSLSHSPGKGGGGSGGGGSGGGGSGGGGSGGGGSMVFRPGGGDMRDNWRSELYKYKVIKIEPLGIAPTKAKRRVVQREKRQARQLLSGIVQQQNNLLRAIEAQQHLLQLTVWGIKQLQARVLAVERYLRDQQLLGIWGCSGKLICTTAVPWNASWSNKSLEDIWDNMTWMQWEREIDNYTNTIYTLLEESQNQQEKNEQELL

SEQ ID NO: 104 - protein, 684 aa, Synthetic
MYRMQLLSCIALSLALVTNSMVFRPGGGDMRDNWRSELYKYKVIKIEPLGIAPTKAKRRVVQREKRQARQLLSGIVQQQNNLLRAIEAQQHLLQLTVWGIKQLQARVLAVERYLRDQQLLGIWGCSGKLICTTAVPWNASWSNKSLEDIWDNMTWMQWEREIDNYTNTIYTLLEESQNQQEKNEQELLGGGGSGGGGSGGGGSGGGGSGGGGSVPEVSSVFIFPPKPKDVLTITLTPKVTCVVVDISKDDPEVQFSWFVDDVEVHTAQTQPREEQFNSTFRSVSELPIMHQDWLNGKEFKCRVNSAAFPAPIEKTISKTKGRPKAPQVYTIPPPKEQMAKDKVSLTCMITDFFPEDITVEWQWNGQPAENYKNTQPIMDTDGSYFVYSKLNVQKSNWEAGNTFTCSVLHEGLHNHHTEKSLSHSPGKGGGGSGGGGSGGGGSGGGGSGGGGSMPIVQNLQGQMVHQAISPRTLNAWVKVVEEKAFSPEVIPMFSALSAGATPAAANTALNTAGGHQAAMQMLKETINEEAAEWDRVHPVHAGPAAPGAAAAPAGSAAAGTTSTAQAQAGWATNNPPAPAGAAAAAWIAAGANAAVAAYSPTSALDAAAGPAAPFRAAAAAFYATLAAAQASQDVKNWMTATAAAANANPACKTILKALGPAATLEEMMTACQGVGGPGHKARVL

SEQ ID NO: 105 - protein, 684 aa, Synthetic
MYRMQLLSCIALSLALVTNSMPIVQNLQGQMVHQAISPRTLNAWVKVVEEKAFSPEVIPMFSALSAGATPAAANTALNTAGGHQAAMQMLKETINEEAAEWDRVHPVHAGPAAPGAAAAPAGSAAAGTTSTAQAQAGWATNNPPAPAGAAAAAWIAAGANAAVAAYSPTSALDAAAGPAAPFRAAAAAFYATLAAAQASQDVKNWMTATAAAANANPACKTILKALGPAATLEEMMTACQGVGGPGHKARVLGGGGSGGGGSGGGGSGGGGSGGGGSVPEVSSVFIFPPKPKDVLTITLTPKVTCVVVDISKDDPEVQFSWFVDDVEVHTAQTQPREEQFNSTFRSVSELPIMHQDWLNGKEFKCRVNSAAFPAPIEKTISKTKGRPKAPQVYTIPPPKEQMAKDKVSLTCMITDFFPEDITVEWQWNGQPAENYKNTQPIMDTDGSYFVYSKLNVQKSNWEAGNTFTCSVLHEGLHNHHTEKSLSHSPGKGGGGSGGGGSGGGGSGGGGSGGGGSMVFRPGGGDMRDNWRSELYKYKVIKIEPLGIAPTKAKRRVVQREKRQARQLLSGIVQQQNNLLRAIEAQQHLLQLTVWGIKQLQARVLAVERYLRDQQLLGIWGCSGKLICTTAVPWNASWSNKSLEDIWDNMTWMQWEREIDNYTNTIYTLLEESQNQQEKNEQELL

SEQ ID NO: 106 - protein, 800 aa, Synthetic
MYRMQLLSCIALSLALVTNSAVGIGAVFLGFLGAAGSTMGAASMTLTVQARNLLSGIVQQQSNLLRAPEAQQHLLKLTVWGIKQLQARVLAVERYLRDQQLLGIWGCSGKLICCTNVPWNSSWSNRNLSEIWDNMTWLQWDKEISNYTQIIYGLLEESQNQQEKNEQDLLALDKWASLWNWFDITNWLWYIQAPNLLGGPSVFIFPPKIKDVLMISLSPIVTCVVVDVSEDDPDVQISWFVNNVEVHTAQTQTHREDYNSTLRVVSALPIQHQDWMSGKEFKCKVNNKDLPAPIERTISKPKGSVRAPQVYVLPPPEEEMTKKQVTLTCMVTDFMPEDIYVEWTNNGKTELNYKNTEPVLDSDGSYFMYSKLRVEKKNWVERNSYSCSVVHEGLHNHHTTKSFSRTPGKAEAAAKEAAAKAAWEDADTTLFCASDAKAYSTEKHNVWATHACVPTDPDPQEIPLENVTENFNMWKNNMVEQMHEDIISLWDESLKPCVMLTGGSTIKQACPKVTFEPIPIHYCAPAGFAILKCRDEDFNGTGPCKNVSTVQCTHGIKPVVSTQLLLNGSLAKGDIVIRSENLTNNAKVIIVQLNEPVQIVCIRPNNGGSGSGGDIRQAHCNVTRSRWNKTLQEVKEQLWKIFNKTTNITFNNTIFNSPAGGDLEITTHSFNCGGEFFYCNTSDLFNETNLSANHTDTNENITLQCRIKQIVRMWQRVGQAMYAPPIAGNITCISNITGLLLTRDGVNDTHDKENETFRPTGGDMRDNWRSELYKYKVVRIEINFANSTGGDLEITTHSFN

SEQ ID NO: 107 - protein, 226 aa, Synthetic
VPRDCGCKPCICTVPEVSSVFIFPPKPKDVLTITLTPKVTCVVVDISKDDPEVQFSWFVDDVEVHTAQTQPREEQFNSTFRSVSELPIMHQDWLNGKEFKCRVNSAAFPAPIEKTISKTKGRPKAPQVYTIPPPKEQMAKDKVSLTCMITDFFPEDITVEWQWNGQPAENYKNTQPIMDTDGSYFVYSKLNVQKSNWEAGNTFTCSVLHEGLHNHHTEKSLSHSPG

SEQ ID NO: 108 - protein, 13 aa, Synthetic
VPRDCGCKPCICT

SEQ ID NO: 109 - protein, 15 aa, Synthetic
GGGGSGGGGSGGGGS

SEQ ID NO: 110 - protein, 25 aa, Synthetic
GGGGSGGGGSGGGGSGGGGSGGGGS

SEQ ID NO: 111 - protein, 5 aa, Synthetic
GGGPS